European Patent Specification EP 3 322 797 B1, published November 29, 2023. Title: IMPROVING SEQUENCE-SPECIFIC ANTIMICROBIALS BY BLOCKING DNA REPAIR. Applicant: INSTITUT PASTEUR ELIGO BIOSCIENCE. The sequence listing filed with the application follows.

SEQUENCE LISTING (72 sequences)

SEQ ID NO: 1 - DNA, 36 bp, Artificial
  repeat sequence
gtttttgtactctcaagatttaagtaactgtacaac

SEQ ID NO: 2 - DNA, 36 bp, Artificial
  repeat sequence
gatataaacctaattacctcgagaggggacggaaac

SEQ ID NO: 3 - DNA, 36 bp, Artificial
  repeat sequence
gttttggaaccattcgaaacaacacagctctaaaac

SEQ ID NO: 4 - DNA, 36 bp, Artificial
  repeat sequence
gttttagagctatgctgttttgaatggtcccaaaac

SEQ ID NO: 5 - DNA, 32 bp, Artificial
  repeat sequence
atttcaatccactcacccatgaagggtgagac

SEQ ID NO: 6 - DNA, 37 bp, Artificial
  repeat sequence
gtttcagtagctagattatttgatatactgctgttag

SEQ ID NO: 7 - DNA, 36 bp, Artificial
  repeat sequence
aatcagagaataccccgtataaaaggggacgagaac

SEQ ID NO: 8 - DNA, 28 bp, Artificial
  repeat sequence
gttcactgccgcacaggcagcttagaaa

SEQ ID NO: 9 - DNA, 37 bp, Artificial
  repeat sequence
ggttgtagctccctttctcatttcgcagtgctacaat

SEQ ID NO: 10 - DNA, 28 bp, Artificial
  repeat sequence
ccggattcccgcctgcgcgggaatgacg

SEQ ID NO: 11 - DNA, 5120 bp, Artificial
  pLC13
atcgatgcataatgtgcctgtcaaatggacgaagcagggattctgcaaaccctatgctactccgtcaagccgtcaattgtctgattcgttaccaattatgacaacttgacggctacatcattcactttttcttcacaaccggcacggaactcgctcgggctggccccggtgcattttttaaatacccgcgagaaatagagttgatcgtcaaaaccaacattgcgaccgacggtggcgataggcatccgggtggtgctcaaaagcagcttcgcctggctgatacgttggtcctcgcgccagcttaagacgctaatccctaactgctggcggaaaagatgtgacagacgcgacggcgacaagcaaacatgctgtgcgacgctggcgatatcaaaattgctgtctgccaggtgatcgctgatgtactgacaagcctcgcgtacccgattatccatcggtggatggagcgactcgttaatcgcttccatgcgccgcagtaacaattgctcaagcagatttatcgccagcagctccgaatagcgcccttccccttgcccggcgttaatgatttgcccaaacaggtcgctgaaatgcggctggtgcgcttcatccgggcgaaagaaccccgtattggcaaatattgacggccagttaagccattcatgccagtaggcgcgcggacgaaagtaaacccactggtgataccattcgcgagcctccggatgacgaccgtagtgatgaatctctcctggcgggaacagcaaaatatcacccggtcggcaaacaaattctcgtccctgatttttcaccaccccctgaccgcgaatggtgagattgagaatataacctttcattcccagcggtcggtcgataaaaaaatcgagataaccgttggcctcaatcggcgttaaacccgccaccagatgggcattaaacgagtatcccggcagcaggggatcattttgcgcttcagccatacttttcatactcccgccattcagagaagaaaccaattgtccatattgcatcagacattgccgtcactgcgtcttttactggctcttctcgctaaccaaaccggtaaccccgcttattaaaagcattctgtaacaaagcgggaccaaagccatgacaaaaacgcgtaacaaaagtgtctataatcacggcagaaaagtccacattgattatttgcacggcgtcacactttgctatgccatagcatttttatccataagattagcggatcctacctgacgctttttatcgcaactctctactgtttctccatacccgtttttttgggctagcgaattcgagctcggtaactttaagaaggagatataccatggctaaaccagcaaaacgtatcaagagtgccgcagcggcttatgtgccacaaaaccgcgatgcggtgattaccgatattaaacgcatcggggatttacagcgcgaagcatcacgtctggaaacggaaatgaatgatgccatcgcggaaattacggagaaatttgcggcccggattgcaccgattaaaaccgatattgaaaccctttcaaaaggcgttcagggatggtgtgaagcgaaccgcgacgaactgacgaacggcggcaaagtgaagacggcgaatcttgtcaccggtgatgtatcgtggcgggtccgtccaccatcagtaagtattcgtggtatggatgcagtgatggaaacgctggagcgtcttggcctgcaacgctttattcgcacgaagcaggaaatcaacaaggaagcgattttactggaaccgaaagcggtcgcaggcgttgccggaattacagttaaatcaggcattgaggatttttctattattccatttgaacaggaagccggtatttaattggctgttttggcggatgagagaagattttcagcctgatacagattaaatcagaacgcagaagcggtctgataaaacagaatttgcctggcggcagtagcgcggtggtcccacctgaccccatgccgaactcagaagtgaaacgccgtagcgccgatggtagtgtggggtctccccatgcgagagtagggaactgccaggcatcaaataaaacgaaaggctcagtcgaaagactgggcctttcgttttatctgttgtttgtcggtgaacgctctcctgagtaggacaaatccgccgggagcggatttgaacgttgcgaagcaacggcccggagggtggcgggcaggacgcccgccataaactgccaggcatcaaattaagcagaaggccatcctgacggatggcctttttgcgtttctacaaactcttttgtttatttttctaaatacattcaaatatgtatccgctcatgagacaataaccctgataaatgcttcaataatattgaaaaaggaagagtatgagtattcaacatttccgtgtcgcccttattcccttttttgcggcattttgccttcctgtttttgctcacccagaaacgctggtgaaagtaaaagatgctgaagatcagttgggtgcacgagtgggttacatcgaactggatctcaacagcggtaagatccttgagagttttcgccccgaagaacgttttccaatgatgagcacttttaaagttctgctatgtggcgcggtattatcccgtgttgacgccgggcaagagcaactcggtcgccgcatacactattctcagaatgacttggttgagtactcaccagtcacagaaaagcatcttacggatggcatgacagtaagagaattatgcagtgctgccataaccatgagtgataacactgcggccaacttacttctgacaacgatcggaggaccgaaggagctaaccgcttttttgcacaacatgggggatcatgtaactcgccttgatcgttgggaaccggagctgaatgaagccataccaaacgacgagcgtgacaccacgatgcctgcagcaatggcaacaacgttgcgcaaactattaactggcgaactacttactctagcttcccggcaacaattaatagactggatggaggcggataaagttgcaggaccacttctgcgctcggcccttccggctggctggtttattgctgataaatctggagccggtgagcgtgggtctcgcggtatcattgcagcactggggccagatggtaagccctcccgtatcgtagttatctacacgacggggagtcaggcaactatggatgaacgaaatagacagatcgctgagataggtgcctcactgattaagcattggtaactgtcagaccaagtttactcatatatactttagattgatttacgcgccctgtagcggcgcattaagcgcggcgggtgtggtggttacgcgcagcgtgaccgctacacttgccagcgccctagcgcccgctcctttcgctttcttcccttcctttctcgccacgttcgccggctttccccgtcaagctctaaatcgggggctccctttagggttccgatttagtgctttacggcacctcgaccccaaaaaacttgatttgggtgatggttcacgtagtgggccatcgccctgatagacggtttttcgccctttgacgttggagtccacgttctttaatagtggactcttgttccaaacttgaacaacactcaaccctatctcgggctattcttttgatttataagggattttgccgatttcggcctattggttaaaaaatgagctgatttaacaaaaatttaacgcgaattttaacaaaatattaacgtttacaatttaaaaggatctaggtgaagatcctttttgataatctcatgaccaaaatcccttaacgtgagttttcgttccactgagcgtcagaccccgtagaaaagatcaaaggatcttcttgagatcctttttttctgcgcgtaatctgctgcttgcaaacaaaaaaaccaccgctaccagcggtggtttgtttgccggatcaagagctaccaactctttttccgaaggtaactggcttcagcagagcgcagataccaaatactgtccttctagtgtagccgtagttaggccaccacttcaagaactctgtagcaccgcctacatacctcgctctgctaatcctgttaccagtggctgctgccagtggcgataagtcgtgtcttaccgggttggactcaagacgatagttaccggataaggcgcagcggtcgggctgaacggggggttcgtgcacacagcccagcttggagcgaacgacctacaccgaactgagatacctacagcgtgagctatgagaaagcgccacgcttcccgaagggagaaaggcggacaggtatccggtaagcggcagggtcggaacaggagagcgcacgagggagcttccagggggaaacgcctggtatctttatagtcctgtcgggtttcgccacctctgacttgagcgtcgatttttgtgatgctcgtcaggggggcggagcctatggaaaaacgccagcaacgcggcctttttacggttcctggccttttgctggccttttgctcacatgttctttcctgcgttatcccctgattctgtggataaccgtattaccgcctttgagtgagctgataccgctcgccgcagccgaacgaccgagcgcagcgagtcagtgagcgaggaagcggaagagcgcctgatgcggtattttctccttacgcatctgtgcggtatttcacaccgcatatggtgcactctcagtacaatctgctctgatgccgcatagttaagccagtatacactccgctatcgctacgtgactgggtcatggctgcgccccgacacccgccaacacccgctgacgcgccctgacgggcttgtctgctcccggcatccgcttacagacaagctgtgaccgtctccgggagctgcatgtgtcagaggttttcaccgtcatcaccgaaacgcgcgaggcagcaaggagatggcgcccaacagtcccccggccacggggcctgccaccatacccacgccgaaacaagcgctcatgagcccgaagtggcgagcccgatcttccccatcggtgatgtcggcgatataggcgccagcaaccgcacctgtggcgccggtgatgccggccacgatgcgtccggcgtagaggatctgctcatgtttgacagcttatc

SEQ ID NO: 12 - DNA, 30 bp, Artificial
  primer LC2
ccttcttaaagttaccgagctcgaattcgc

SEQ ID NO: 13 - DNA, 60 bp, Artificial
  primer LC296
tatattttaggaattctaaagatctttgacagctagctcagtcctaggtataatactagt

SEQ ID NO: 14 - DNA, 39 bp, Artificial
  primer LC397
atccgccaaaacagccaattaaataccggcttcctgttc

SEQ ID NO: 15 - DNA, 61 bp, Artificial
  primer LC398
gcgaattcgagctcggtaactttaagaaggagatataccatggctaaaccagcaaaacgta

SEQ ID NO: 16 - DNA, 30 bp, Artificial
  CRISPR spacer LacZ1
tcactggccgtcgttttacaacgtcgtgac

SEQ ID NO: 17 - DNA, 30 bp, Artificial
  CRISPR spacer LacZ2
ccattacggtcaatccgccgtttgttccca

SEQ ID NO: 18 - DNA, 30 bp, Artificial
  CRISPR spacer rpsL
tactttacgcagcgcggagttcggtttttt

SEQ ID NO: 19 - DNA, 30 bp, Artificial
  CRISPR spacer mhpR
ggaattaatcgaaatgttagcctcccgccc

SEQ ID NO: 20 - DNA, 30 bp, Artificial
  CRISPR spacer tsuB
taaggtcttcgttcagggcatagaccttaa

SEQ ID NO: 21 - DNA, 30 bp, Artificial
  CRISPR spacer wcaH
ttttctcgctgagaagcgtaccggagtacc

SEQ ID NO: 22 - DNA, 30 bp, Artificial
  CRISPR spacer irhA
attccgctgcgcagtaccagtgtgttggcg

SEQ ID NO: 23 - DNA, 30 bp, Artificial
  CRISPR spacer eamB
cagcggtacaccttttgagttgggcggggg

SEQ ID NO: 24 - DNA, 30 bp, Artificial
  CRISPR spacer speA
agcagaacgtctgaatgtcgttcctcgtct

SEQ ID NO: 25 - DNA, 30 bp, Artificial
  CRISPR spacer garD
cgtggtggggctgaatcatttgtacggttg

SEQ ID NO: 26 - DNA, 30 bp, Artificial
  CRISPR spacer treF
gtaccgcgatttacgcgcgggggcggcctc

SEQ ID NO: 27 - DNA, 30 bp, Artificial
  CRISPR spacer yfaP
attcgtgcacgtttacggctggttctctcg

SEQ ID NO: 28 - DNA, 30 bp, Artificial
  CRISPR spacer ada
ggtgcgttacgcgctggctgattgtgagct

SEQ ID NO: 29 - DNA, 33 bp, Artificial
  primer B299
catgaattcaactcaacaagtctcagtgtgctg

SEQ ID NO: 30 - DNA, 40 bp, Artificial
  primer LC34
tttaggcgctgccatcttaagacgaaagggcctcgtgata

SEQ ID NO: 31 - DNA, 63 bp, Artificial
  primer LC35
ttcagcacactgagacttgttgagttgaattcatgagtattaagtattgttttatggctgata

SEQ ID NO: 32 - DNA, 40 bp, Artificial
  primer LC36
tatcacgaggccctttcgtcttaagatggcagcgcctaaa

SEQ ID NO: 33 - DNA, 37 bp, Artificial
  primer LC41
tgcagcgcgatcgtaatcaggatcccatggtacgcgt

SEQ ID NO: 34 - DNA, 37 bp, Artificial
  primer LC42
acagaacttaatgggcccgaagacgaaagggcctcgt

SEQ ID NO: 35 - DNA, 40 bp, Artificial
  primer LC37
tccgccgtttgttcccacgtagaatccgacgggttgttac

SEQ ID NO: 36 - DNA, 40 bp, Artificial
  primer LC38
gtaacaacccgtcggattctacgtgggaacaaacggcgga

SEQ ID NO: 37 - DNA, 37 bp, Artificial
  primer LC39
acgaggccctttcgtcttcgggcccattaagttctgt

SEQ ID NO: 38 - DNA, 37 bp, Artificial
  primer LC40
acgcgtaccatgggatcctgattacgatcgcgctgca

SEQ ID NO: 39 - DNA, 19 bp, Artificial
  primer LC191
gtctagggcggcggatttg

SEQ ID NO: 40 - DNA, 22 bp, Artificial
  primer LC192
cgctctcctgagtaggacaaat

SEQ ID NO: 41 - DNA, 36 bp, Artificial
  primer LC193
acaattgaataccgatcggcctcgtgatacgcctat

SEQ ID NO: 42 - DNA, 42 bp, Artificial
  primer LC194
ataggcgtatcacgaggccgatcggtattcaattgtgcccaa

SEQ ID NO: 43 - DNA, 41 bp, Artificial
  primer LC195
caggggctggattgattatgagtaaaggagaagaacttttc

SEQ ID NO: 44 - DNA, 38 bp, Artificial
  primer LC196
ttcttctcctttactcataatcaatccagcccctgtga

SEQ ID NO: 45 - DNA, 42 bp, Artificial
  primer LC95
ctccgacgccgaacccatacaacctccttagtacatcaagca

SEQ ID NO: 46 - DNA, 58 bp, Artificial
  primer LC96
gcaggacgcccgccataaactgccaggaattggggatcggggggttccgcgcacattt

SEQ ID NO: 47 - DNA, 58 bp, Artificial; identical to SEQ ID NO: 46
  primer LC94

SEQ ID NO: 48 - DNA, 59 bp, Artificial
  primer LC98
agtttaggttaggcgccatgcatctcgaggcatgcctgcatcattcgcgcaccacctca

SEQ ID NO: 49 - DNA, 42 bp, Artificial
  primer LC93
cgtccaaatggctcgcatacaacctccttagtacatcaagca

SEQ ID NO: 50 - DNA, 42 bp, Artificial
  primer LC92
tgcttgatgtactaaggaggttgtatgcgagccatttggacg

SEQ ID NO: 51 - DNA, 58 bp, Artificial
  primer LC97
agtttaggttaggcgccatgcatctcgaggcatgcctgcatcacggaggcgttgggac

SEQ ID NO: 52 - DNA, 64 bp, Artificial
  primer LC100
gcaggacgcccgccataaactgccaggaattggggatcggttaagacccactttcacatttaag

SEQ ID NO: 53 - DNA, 59 bp, Artificial
  primer LC101
agtttaggttaggcgccatgcatctcgaggcatgcctgcatataaacgcagaaaggccc

SEQ ID NO: 54 - DNA, 18 bp, Artificial
  primer LC33
gactggaaagcgggcagt

SEQ ID NO: 55 - DNA, 20 bp, Artificial
  primer LC47
cgcacgatagagattcggga

SEQ ID NO: 56 - DNA, 20 bp, Artificial
  primer LC80
tcaggcgggatgaagatgat

SEQ ID NO: 57 - DNA, 21 bp, Artificial
  primer LC153
gctgggatacgctggtgttta

SEQ ID NO: 58 - DNA, 19 bp, Artificial
  primer LC154
cacagcgcaaggacgttga

SEQ ID NO: 59 - DNA, 18 bp, Artificial
  primer LC155
acacaacatgacgggctt

SEQ ID NO: 60 - DNA, 9326 bp, Artificial
  pCas9 (pCas9-a)
  gene (219)..(8886): gene cat - positions are given on the complementary strand : complement (8886..219)
  promoter (220)..(322): cat promoter - positions are given on the complementary strand : complement (220..322)
  rep_origin (848)..(1393): p15A ori - positions are given on the complementary strand : complement (848..1393)
  promoter (1505)..(1533): tet promoter
  misc_feature (1844)..(2014): tracrRNA sequence of S. p (Zhangfeng) - positions are given on the complementary strand : complement (1844..2014)
  misc_feature (1846)..(1932): tracrRNA sequence of S. p (Zhangfeng)
  gene (2225)..(6331): Cas9 (Csn1) endonuclease from the streptococcus pyogenes Type II CRISPR/Cas system
  misc_feature (6484)..(6519): repeat
  misc_feature (6550)..(6585): repeat
gaattccggatgagcattcatcaggcgggcaagaatgtgaataaaggccggataaaacttgtgcttatttttctttacggtctttaaaaaggccgtaatatccagctgaacggtctggttataggtacattgagcaactgactgaaatgcctcaaaatgttctttacgatgccattgggatatatcaacggtggtatatccagtgatttttttctccattttagcttccttagctcctgaaaatctcgataactcaaaaaatacgcccggtagtgatcttatttcattatggtgaaagttggaacctcttacgtgccgatcaacgtctcattttcgccaaaagttggcccagggcttcccggtatcaacagggacaccaggatttatttattctgcgaagtgatcttccgtcacaggtatttattcggcgcaaagtgcgtcgggtgatgctgccaacttactgatttagtgtatgatggtgtttttgaggtgctccagtggcttctgtttctatcagctgtccctcctgttcagctactgacggggtggtgcgtaacggcaaaagcaccgccggacatcagcgctagcggagtgtatactggcttactatgttggcactgatgagggtgtcagtgaagtgcttcatgtggcaggagaaaaaaggctgcaccggtgcgtcagcagaatatgtgatacaggatatattccgcttcctcgctcactgactcgctacgctcggtcgttcgactgcggcgagcggaaatggcttacgaacggggcggagatttcctggaagatgccaggaagatacttaacagggaagtgagagggccgcggcaaagccgtttttccataggctccgcccccctgacaagcatcacgaaatctgacgctcaaatcagtggtggcgaaacccgacaggactataaagataccaggcgtttccccctggcggctccctcgtgcgctctcctgttcctgcctttcggtttaccggtgtcattccgctgttatggccgcgtttgtctcattccacgcctgacactcagttccgggtaggcagttcgctccaagctggactgtatgcacgaaccccccgttcagtccgaccgctgcgccttatccggtaactatcgtcttgagtccaacccggaaagacatgcaaaagcaccactggcagcagccactggtaattgatttagaggagttagtcttgaagtcatgcgccggttaaggctaaactgaaaggacaagttttggtgactgcgctcctccaagccagttacctcggttcaaagagttggtagctcagagaaccttcgaaaaaccgccctgcaaggcggttttttcgttttcagagcaagagattacgcgcagaccaaaacgatctcaagaagatcatcttattaatcagataaaatatttctagatttcagtgcaatttatctcttcaaatgtagcacctgaagtcagccccatacgatataagttgtaattctcatgtttgacagcttatcatcgataagctttaatgcggtagtttatcacagttaaattgctaacgcagtcaggcaccgtgtatgaaatctaacaatgcgctcatcgtcatcctcggcaccgtcaccctggatgctgtaggcataggcttggttatgccggtactgccgggcctcttgcgggattacgaaatcatcctgtggagcttagtaggtttagcaagatggcagcgcctaaatgtagaatgataaaaggattaagagattaatttccctaaaaatgataaaacaagcgttttgaaagcgcttgtttttttggtttgcagtcagagtagaatagaagtatcaaaaaaagcaccgactcggtgccactttttcaagttgataacggactagccttattttaacttgctatgctgttttgaatggttccaacaagattattttataacttttataacaaataatcaaggagaaattcaaagaaatttatcagccataaaacaatacttaatactatagaatgataacaaaataaactactttttaaaagaattttgtgttataatctatttattattaagtattgggtaatattttttgaagagatattttgaaaaagaaaaattaaagcatattaaactaatttcggaggtcattaaaactattattgaaatcatcaaactcattatggatttaatttaaactttttattttaggaggcaaaaatggataagaaatactcaataggcttagatatcggcacaaatagcgtcggatgggcggtgatcactgatgaatataaggttccgtctaaaaagttcaaggttctgggaaatacagaccgccacagtatcaaaaaaaatcttataggggctcttttatttgacagtggagagacagcggaagcgactcgtctcaaacggacagctcgtagaaggtatacacgtcggaagaatcgtatttgttatctacaggagattttttcaaatgagatggcgaaagtagatgatagtttctttcatcgacttgaagagtcttttttggtggaagaagacaagaagcatgaacgtcatcctatttttggaaatatagtagatgaagttgcttatcatgagaaatatccaactatctatcatctgcgaaaaaaattggtagattctactgataaagcggatttgcgcttaatctatttggccttagcgcatatgattaagtttcgtggtcattttttgattgagggagatttaaatcctgataatagtgatgtggacaaactatttatccagttggtacaaacctacaatcaattatttgaagaaaaccctattaacgcaagtggagtagatgctaaagcgattctttctgcacgattgagtaaatcaagacgattagaaaatctcattgctcagctccccggtgagaagaaaaatggcttatttgggaatctcattgctttgtcattgggtttgacccctaattttaaatcaaattttgatttggcagaagatgctaaattacagctttcaaaagatacttacgatgatgatttagataatttattggcgcaaattggagatcaatatgctgatttgtttttggcagctaagaatttatcagatgctattttactttcagatatcctaagagtaaatactgaaataactaaggctcccctatcagcttcaatgattaaacgctacgatgaacatcatcaagacttgactcttttaaaagctttagttcgacaacaacttccagaaaagtataaagaaatcttttttgatcaatcaaaaaacggatatgcaggttatattgatgggggagctagccaagaagaattttataaatttatcaaaccaattttagaaaaaatggatggtactgaggaattattggtgaaactaaatcgtgaagatttgctgcgcaagcaacggacctttgacaacggctctattccccatcaaattcacttgggtgagctgcatgctattttgagaagacaagaagacttttatccatttttaaaagacaatcgtgagaagattgaaaaaatcttgacttttcgaattccttattatgttggtccattggcgcgtggcaatagtcgttttgcatggatgactcggaagtctgaagaaacaattaccccatggaattttgaagaagttgtcgataaaggtgcttcagctcaatcatttattgaacgcatgacaaactttgataaaaatcttccaaatgaaaaagtactaccaaaacatagtttgctttatgagtattttacggtttataacgaattgacaaaggtcaaatatgttactgaaggaatgcgaaaaccagcatttctttcaggtgaacagaagaaagccattgttgatttactcttcaaaacaaatcgaaaagtaaccgttaagcaattaaaagaagattatttcaaaaaaatagaatgttttgatagtgttgaaatttcaggagttgaagatagatttaatgcttcattaggtacctaccatgatttgctaaaaattattaaagataaagattttttggataatgaagaaaatgaagatatcttagaggatattgttttaacattgaccttatttgaagatagggagatgattgaggaaagacttaaaacatatgctcacctctttgatgataaggtgatgaaacagcttaaacgtcgccgttatactggttggggacgtttgtctcgaaaattgattaatggtattagggataagcaatctggcaaaacaatattagattttttgaaatcagatggttttgccaatcgcaattttatgcagctgatccatgatgatagtttgacatttaaagaagacattcaaaaagcacaagtgtctggacaaggcgatagtttacatgaacatattgcaaatttagctggtagccctgctattaaaaaaggtattttacagactgtaaaagttgttgatgaattggtcaaagtaatggggcggcataagccagaaaatatcgttattgaaatggcacgtgaaaatcagacaactcaaaagggccagaaaaattcgcgagagcgtatgaaacgaatcgaagaaggtatcaaagaattaggaagtcagattcttaaagagcatcctgttgaaaatactcaattgcaaaatgaaaagctctatctctattatctccaaaatggaagagacatgtatgtggaccaagaattagatattaatcgtttaagtgattatgatgtcgatcacattgttccacaaagtttccttaaagacgattcaatagacaataaggtcttaacgcgttctgataaaaatcgtggtaaatcggataacgttccaagtgaagaagtagtcaaaaagatgaaaaactattggagacaacttctaaacgccaagttaatcactcaacgtaagtttgataatttaacgaaagctgaacgtggaggtttgagtgaacttgataaagctggttttatcaaacgccaattggttgaaactcgccaaatcactaagcatgtggcacaaattttggatagtcgcatgaatactaaatacgatgaaaatgataaacttattcgagaggttaaagtgattaccttaaaatctaaattagtttctgacttccgaaaagatttccaattctataaagtacgtgagattaacaattaccatcatgcccatgatgcgtatctaaatgccgtcgttggaactgctttgattaagaaatatccaaaacttgaatcggagtttgtctatggtgattataaagtttatgatgttcgtaaaatgattgctaagtctgagcaagaaataggcaaagcaaccgcaaaatatttcttttactctaatatcatgaacttcttcaaaacagaaattacacttgcaaatggagagattcgcaaacgccctctaatcgaaactaatggggaaactggagaaattgtctgggataaagggcgagattttgccacagtgcgcaaagtattgtccatgccccaagtcaatattgtcaagaaaacagaagtacagacaggcggattctccaaggagtcaattttaccaaaaagaaattcggacaagcttattgctcgtaaaaaagactgggatccaaaaaaatatggtggttttgatagtccaacggtagcttattcagtcctagtggttgctaaggtggaaaaagggaaatcgaagaagttaaaatccgttaaagagttactagggatcacaattatggaaagaagttcctttgaaaaaaatccgattgactttttagaagctaaaggatataaggaagttaaaaaagacttaatcattaaactacctaaatatagtctttttgagttagaaaacggtcgtaaacggatgctggctagtgccggagaattacaaaaaggaaatgagctggctctgccaagcaaatatgtgaattttttatatttagctagtcattatgaaaagttgaagggtagtccagaagataacgaacaaaaacaattgtttgtggagcagcataagcattatttagatgagattattgagcaaatcagtgaattttctaagcgtgttattttagcagatgccaatttagataaagttcttagtgcatataacaaacatagagacaaaccaatacgtgaacaagcagaaaatattattcatttatttacgttgacgaatcttggagctcccgctgcttttaaatattttgatacaacaattgatcgtaaacgatatacgtctacaaaagaagttttagatgccactcttatccatcaatccatcactggtctttatgaaacacgcattgatttgagtcagctaggaggtgactgaagtatattttagatgaagattatttcttaataactaaaaatatggtataatactcttaataaatgcagtaatacaggggcttttcaagactgaagtctagctgagacaaatagtgcgattacgaaattttttagacaaaaatagtctacgaggttttagagctatgctgttttgaatggtcccaaaactgagaccagtctcggaagctcaaaggtctcgttttagagctatgctgttttgaatggtcccaaaacttcagcacactgagacttgttgagttccatgttttagagctatgctgttttgaatggactccattcaacattgccgatgataacttgagaaagagggttaataccagcagtcggataccttcctattctttctgttaaagcgttttcatgttataataggcaaaagaagagtagtgtgatcgtccattccgacagcatcgccagtcactatggcgtgctgctagcgctatatgcgttgatgcaatttctatgcgcacccgttctcggagcactgtccgaccgctttggccgccgcccagtcctgctcgcttcgctacttggagccactatcgactacgcgatcatggcgaccacacccgtcctgtggatcctctacgccggacgcatcgtggccggcatcaccggcgccacaggtgcggttgctggcgcctatatcgccgacatcaccgatggggaagatcgggctcgccacttcgggctcatgagcgcttgtttcggcgtgggtatggtggcaggccccgtggccgggggactgttgggcgccatctccttgcatgcaccattccttgcggcggcggtgctcaacggcctcaacctactactgggctgcttcctaatgcaggagtcgcataagggagagcgtcgaccgatgcccttgagagccttcaacccagtcagctccttccggtgggcgcggggcatgactatcgtcgccgcacttatgactgtcttctttatcatgcaactcgtaggacaggtgccggcagcgctctgggtcattttcggcgaggaccgctttcgctggagcgcgacgatgatcggcctgtcgcttgcggtattcggaatcttgcacgccctcgctcaagccttcgtcactggtcccgccaccaaacgtttcggcgagaagcaggccattatcgccggcatggcggccgacgcgctgggctacgtcttgctggcgttcgcgacgcgaggctggatggccttccccattatgattcttctcgcttccggcggcatcgggatgcccgcgttgcaggccatgctgtccaggcaggtagatgacgaccatcagggacagcttcaaggatcgctcgcggctcttaccagcctaacttcgatcattggaccgctgatcgtcacggcgatttatgccgcctcggcgagcacatggaacgggttggcatggattgtaggcgccgccctataccttgtctgcctccccgcgttgcgtcgcggtgcatggagccgggccacctcgacctgaatggaagccggcggcacctcgctaacggattcaccactccaagaattggagccaatcaattcttgcggagaactgtgaatgcgcaaaccaacccttggcagaacatatccatcgcgtccgccatctccagcagccgcacgcggcgcatctcgggcagcgttgggtcctggccacgggtgcgcatgatcgtgctcctgtcgttgaggacccggctaggctggcggggttgccttactggttagcagaatgaatcaccgatacgcgagcgaacgtgaagcgactgctgctgcaaaacgtctgcgacctgagcaacaacatgaatggtcttcggtttccgtgtttcgtaaagtctggaaacgcggaagtcccctacgtgctgctgaagttgcccgcaacagagagtggaaccaaccggtgataccacgatactatgactgagagtcaacgccatgagcggcctcatttcttattctgagttacaacagtccgcaccgctgtccggtagctccttccggtgggcgcggggcatgactatcgtcgccgcacttatgactgtcttctttatcatgcaactcgtaggacaggtgccggcagcgcccaacagtcccccggccacggggcctgccaccatacccacgccgaaacaagcgccctgcaccattatgttccggatctgcatcgcaggatgctgctggctaccctgtggaacacctacatctgtattaacgaagcgctaaccgtttttatcaggctctgggaggcagaataaatgatcatatcgtcaattattacctccacggggagagcctgagcaaactggcctcaggcatttgagaagcacacggtcacactgcttccggtagtcaataaaccggtaaaccagcaatagacataagcggctatttaacgaccctgccctgaaccgacgaccgggtcgaatttgctttcgaatttctgccattcatccgcttattatcacttattcaggcgtagcaccaggcgtttaagggcaccaataactgccttaaaaaaattacgccccgccctgccactcatcgcagtactgttgtaattcattaagcattctgccgacatggaagccatcacagacggcatgatgaacctgaatcgccagcggcatcagcaccttgtcgccttgcgtataatatttgcccatggtgaaaacgggggcgaagaagttgtccatattggccacgtttaaatcaaaactggtgaaactcacccagggattggctgagacgaaaaacatattctcaataaaccctttagggaaataggccaggttttcaccgtaacacgccacatcttgcgaatatatgtgtagaaactgccggaaatcgtcgtggtattcactccagagcgatgaaaacgtttcagtttgctcatggaaaacggtgtaacaagggtgaacactatcccatatcaccagctcaccgtctttcattgccatacg

SEQ ID NO: 61 - DNA, 9326 bp, Artificial
  pCas9_LacZ2
  gene (2225)..(6331): product
  misc_feature (6484)..(6519): repeat
  misc_feature (6520)..(6549): CRSIPR target ELZ2
  misc_feature (6550)..(6585): repeat
gaattccggatgagcattcatcaggcgggcaagaatgtgaataaaggccggataaaacttgtgcttatttttctttacggtctttaaaaaggccgtaatatccagctgaacggtctggttataggtacattgagcaactgactgaaatgcctcaaaatgttctttacgatgccattgggatatatcaacggtggtatatccagtgatttttttctccattttagcttccttagctcctgaaaatctcgataactcaaaaaatacgcccggtagtgatcttatttcattatggtgaaagttggaacctcttacgtgccgatcaacgtctcattttcgccaaaagttggcccagggcttcccggtatcaacagggacaccaggatttatttattctgcgaagtgatcttccgtcacaggtatttattcggcgcaaagtgcgtcgggtgatgctgccaacttactgatttagtgtatgatggtgtttttgaggtgctccagtggcttctgtttctatcagctgtccctcctgttcagctactgacggggtggtgcgtaacggcaaaagcaccgccggacatcagcgctagcggagtgtatactggcttactatgttggcactgatgagggtgtcagtgaagtgcttcatgtggcaggagaaaaaaggctgcaccggtgcgtcagcagaatatgtgatacaggatatattccgcttcctcgctcactgactcgctacgctcggtcgttcgactgcggcgagcggaaatggcttacgaacggggcggagatttcctggaagatgccaggaagatacttaacagggaagtgagagggccgcggcaaagccgtttttccataggctccgcccccctgacaagcatcacgaaatctgacgctcaaatcagtggtggcgaaacccgacaggactataaagataccaggcgtttccccctggcggctccctcgtgcgctctcctgttcctgcctttcggtttaccggtgtcattccgctgttatggccgcgtttgtctcattccacgcctgacactcagttccgggtaggcagttcgctccaagctggactgtatgcacgaaccccccgttcagtccgaccgctgcgccttatccggtaactatcgtcttgagtccaacccggaaagacatgcaaaagcaccactggcagcagccactggtaattgatttagaggagttagtcttgaagtcatgcgccggttaaggctaaactgaaaggacaagttttggtgactgcgctcctccaagccagttacctcggttcaaagagttggtagctcagagaaccttcgaaaaaccgccctgcaaggcggttttttcgttttcagagcaagagattacgcgcagaccaaaacgatctcaagaagatcatcttattaatcagataaaatatttctagatttcagtgcaatttatctcttcaaatgtagcacctgaagtcagccccatacgatataagttgtaattctcatgtttgacagcttatcatcgataagctttaatgcggtagtttatcacagttaaattgctaacgcagtcaggcaccgtgtatgaaatctaacaatgcgctcatcgtcatcctcggcaccgtcaccctggatgctgtaggcataggcttggttatgccggtactgccgggcctcttgcgggattacgaaatcatcctgtggagcttagtaggtttagcaagatggcagcgcctaaatgtagaatgataaaaggattaagagattaatttccctaaaaatgataaaacaagcgttttgaaagcgcttgtttttttggtttgcagtcagagtagaatagaagtatcaaaaaaagcaccgactcggtgccactttttcaagttgataacggactagccttattttaacttgctatgctgttttgaatggttccaacaagattattttataacttttataacaaataatcaaggagaaattcaaagaaatttatcagccataaaacaatacttaatactatagaatgataacaaaataaactactttttaaaagaattttgtgttataatctatttattattaagtattgggtaatattttttgaagagatattttgaaaaagaaaaattaaagcatattaaactaatttcggaggtcattaaaactattattgaaatcatcaaactcattatggatttaatttaaactttttattttaggaggcaaaaatggataagaaatactcaataggcttagatatcggcacaaatagcgtcggatgggcggtgatcactgatgaatataaggttccgtctaaaaagttcaaggttctgggaaatacagaccgccacagtatcaaaaaaaatcttataggggctcttttatttgacagtggagagacagcggaagcgactcgtctcaaacggacagctcgtagaaggtatacacgtcggaagaatcgtatttgttatctacaggagattttttcaaatgagatggcgaaagtagatgatagtttctttcatcgacttgaagagtcttttttggtggaagaagacaagaagcatgaacgtcatcctatttttggaaatatagtagatgaagttgcttatcatgagaaatatccaactatctatcatctgcgaaaaaaattggtagattctactgataaagcggatttgcgcttaatctatttggccttagcgcatatgattaagtttcgtggtcattttttgattgagggagatttaaatcctgataatagtgatgtggacaaactatttatccagttggtacaaacctacaatcaattatttgaagaaaaccctattaacgcaagtggagtagatgctaaagcgattctttctgcacgattgagtaaatcaagacgattagaaaatctcattgctcagctccccggtgagaagaaaaatggcttatttgggaatctcattgctttgtcattgggtttgacccctaattttaaatcaaattttgatttggcagaagatgctaaattacagctttcaaaagatacttacgatgatgatttagataatttattggcgcaaattggagatcaatatgctgatttgtttttggcagctaagaatttatcagatgctattttactttcagatatcctaagagtaaatactgaaataactaaggctcccctatcagcttcaatgattaaacgctacgatgaacatcatcaagacttgactcttttaaaagctttagttcgacaacaacttccagaaaagtataaagaaatcttttttgatcaatcaaaaaacggatatgcaggttatattgatgggggagctagccaagaagaattttataaatttatcaaaccaattttagaaaaaatggatggtactgaggaattattggtgaaactaaatcgtgaagatttgctgcgcaagcaacggacctttgacaacggctctattccccatcaaattcacttgggtgagctgcatgctattttgagaagacaagaagacttttatccatttttaaaagacaatcgtgagaagattgaaaaaatcttgacttttcgaattccttattatgttggtccattggcgcgtggcaatagtcgttttgcatggatgactcggaagtctgaagaaacaattaccccatggaattttgaagaagttgtcgataaaggtgcttcagctcaatcatttattgaacgcatgacaaactttgataaaaatcttccaaatgaaaaagtactaccaaaacatagtttgctttatgagtattttacggtttataacgaattgacaaaggtcaaatatgttactgaaggaatgcgaaaaccagcatttctttcaggtgaacagaagaaagccattgttgatttactcttcaaaacaaatcgaaaagtaaccgttaagcaattaaaagaagattatttcaaaaaaatagaatgttttgatagtgttgaaatttcaggagttgaagatagatttaatgcttcattaggtacctaccatgatttgctaaaaattattaaagataaagattttttggataatgaagaaaatgaagatatcttagaggatattgttttaacattgaccttatttgaagatagggagatgattgaggaaagacttaaaacatatgctcacctctttgatgataaggtgatgaaacagcttaaacgtcgccgttatactggttggggacgtttgtctcgaaaattgattaatggtattagggataagcaatctggcaaaacaatattagattttttgaaatcagatggttttgccaatcgcaattttatgcagctgatccatgatgatagtttgacatttaaagaagacattcaaaaagcacaagtgtctggacaaggcgatagtttacatgaacatattgcaaatttagctggtagccctgctattaaaaaaggtattttacagactgtaaaagttgttgatgaattggtcaaagtaatggggcggcataagccagaaaatatcgttattgaaatggcacgtgaaaatcagacaactcaaaagggccagaaaaattcgcgagagcgtatgaaacgaatcgaagaaggtatcaaagaattaggaagtcagattcttaaagagcatcctgttgaaaatactcaattgcaaaatgaaaagctctatctctattatctccaaaatggaagagacatgtatgtggaccaagaattagatattaatcgtttaagtgattatgatgtcgatcacattgttccacaaagtttccttaaagacgattcaatagacaataaggtcttaacgcgttctgataaaaatcgtggtaaatcggataacgttccaagtgaagaagtagtcaaaaagatgaaaaactattggagacaacttctaaacgccaagttaatcactcaacgtaagtttgataatttaacgaaagctgaacgtggaggtttgagtgaacttgataaagctggttttatcaaacgccaattggttgaaactcgccaaatcactaagcatgtggcacaaattttggatagtcgcatgaatactaaatacgatgaaaatgataaacttattcgagaggttaaagtgattaccttaaaatctaaattagtttctgacttccgaaaagatttccaattctataaagtacgtgagattaacaattaccatcatgcccatgatgcgtatctaaatgccgtcgttggaactgctttgattaagaaatatccaaaacttgaatcggagtttgtctatggtgattataaagtttatgatgttcgtaaaatgattgctaagtctgagcaagaaataggcaaagcaaccgcaaaatatttcttttactctaatatcatgaacttcttcaaaacagaaattacacttgcaaatggagagattcgcaaacgccctctaatcgaaactaatggggaaactggagaaattgtctgggataaagggcgagattttgccacagtgcgcaaagtattgtccatgccccaagtcaatattgtcaagaaaacagaagtacagacaggcggattctccaaggagtcaattttaccaaaaagaaattcggacaagcttattgctcgtaaaaaagactgggatccaaaaaaatatggtggttttgatagtccaacggtagcttattcagtcctagtggttgctaaggtggaaaaagggaaatcgaagaagttaaaatccgttaaagagttactagggatcacaattatggaaagaagttcctttgaaaaaaatccgattgactttttagaagctaaaggatataaggaagttaaaaaagacttaatcattaaactacctaaatatagtctttttgagttagaaaacggtcgtaaacggatgctggctagtgccggagaattacaaaaaggaaatgagctggctctgccaagcaaatatgtgaattttttatatttagctagtcattatgaaaagttgaagggtagtccagaagataacgaacaaaaacaattgtttgtggagcagcataagcattatttagatgagattattgagcaaatcagtgaattttctaagcgtgttattttagcagatgccaatttagataaagttcttagtgcatataacaaacatagagacaaaccaatacgtgaacaagcagaaaatattattcatttatttacgttgacgaatcttggagctcccgctgcttttaaatattttgatacaacaattgatcgtaaacgatatacgtctacaaaagaagttttagatgccactcttatccatcaatccatcactggtctttatgaaacacgcattgatttgagtcagctaggaggtgactgaagtatattttagatgaagattatttcttaataactaaaaatatggtataatactcttaataaatgcagtaatacaggggcttttcaagactgaagtctagctgagacaaatagtgcgattacgaaattttttagacaaaaatagtctacgaggttttagagctatgctgttttgaatggtcccaaaacccattacggtcaatccgccgtttgttcccagttttagagctatgctgttttgaatggtcccaaaacttcagcacactgagacttgttgagttccatgttttagagctatgctgttttgaatggactccattcaacattgccgatgataacttgagaaagagggttaataccagcagtcggataccttcctattctttctgttaaagcgttttcatgttataataggcaaaagaagagtagtgtgatcgtccattccgacagcatcgccagtcactatggcgtgctgctagcgctatatgcgttgatgcaatttctatgcgcacccgttctcggagcactgtccgaccgctttggccgccgcccagtcctgctcgcttcgctacttggagccactatcgactacgcgatcatggcgaccacacccgtcctgtggatcctctacgccggacgcatcgtggccggcatcaccggcgccacaggtgcggttgctggcgcctatatcgccgacatcaccgatggggaagatcgggctcgccacttcgggctcatgagcgcttgtttcggcgtgggtatggtggcaggccccgtggccgggggactgttgggcgccatctccttgcatgcaccattccttgcggcggcggtgctcaacggcctcaacctactactgggctgcttcctaatgcaggagtcgcataagggagagcgtcgaccgatgcccttgagagccttcaacccagtcagctccttccggtgggcgcggggcatgactatcgtcgccgcacttatgactgtcttctttatcatgcaactcgtaggacaggtgccggcagcgctctgggtcattttcggcgaggaccgctttcgctggagcgcgacgatgatcggcctgtcgcttgcggtattcggaatcttgcacgccctcgctcaagccttcgtcactggtcccgccaccaaacgtttcggcgagaagcaggccattatcgccggcatggcggccgacgcgctgggctacgtcttgctggcgttcgcgacgcgaggctggatggccttccccattatgattcttctcgcttccggcggcatcgggatgcccgcgttgcaggccatgctgtccaggcaggtagatgacgaccatcagggacagcttcaaggatcgctcgcggctcttaccagcctaacttcgatcattggaccgctgatcgtcacggcgatttatgccgcctcggcgagcacatggaacgggttggcatggattgtaggcgccgccctataccttgtctgcctccccgcgttgcgtcgcggtgcatggagccgggccacctcgacctgaatggaagccggcggcacctcgctaacggattcaccactccaagaattggagccaatcaattcttgcggagaactgtgaatgcgcaaaccaacccttggcagaacatatccatcgcgtccgccatctccagcagccgcacgcggcgcatctcgggcagcgttgggtcctggccacgggtgcgcatgatcgtgctcctgtcgttgaggacccggctaggctggcggggttgccttactggttagcagaatgaatcaccgatacgcgagcgaacgtgaagcgactgctgctgcaaaacgtctgcgacctgagcaacaacatgaatggtcttcggtttccgtgtttcgtaaagtctggaaacgcggaagtcccctacgtgctgctgaagttgcccgcaacagagagtggaaccaaccggtgataccacgatactatgactgagagtcaacgccatgagcggcctcatttcttattctgagttacaacagtccgcaccgctgtccggtagctccttccggtgggcgcggggcatgactatcgtcgccgcacttatgactgtcttctttatcatgcaactcgtaggacaggtgccggcagcgcccaacagtcccccggccacggggcctgccaccatacccacgccgaaacaagcgccctgcaccattatgttccggatctgcatcgcaggatgctgctggctaccctgtggaacacctacatctgtattaacgaagcgctaaccgtttttatcaggctctgggaggcagaataaatgatcatatcgtcaattattacctccacggggagagcctgagcaaactggcctcaggcatttgagaagcacacggtcacactgcttccggtagtcaataaaccggtaaaccagcaatagacataagcggctatttaacgaccctgccctgaaccgacgaccgggtcgaatttgctttcgaatttctgccattcatccgcttattatcacttattcaggcgtagcaccaggcgtttaagggcaccaataactgccttaaaaaaattacgccccgccctgccactcatcgcagtactgttgtaattcattaagcattctgccgacatggaagccatcacagacggcatgatgaacctgaatcgccagcggcatcagcaccttgtcgccttgcgtataatatttgcccatggtgaaaacgggggcgaagaagttgtccatattggccacgtttaaatcaaaactggtgaaactcacccagggattggctgagacgaaaaacatattctcaataaaccctttagggaaataggccaggttttcaccgtaacacgccacatcttgcgaatatatgtgtagaaactgccggaaatcgtcgtggtattcactccagagcgatgaaaacgtttcagtttgctcatggaaaacggtgtaacaagggtgaacactatcccatatcaccagctcaccgtctttcattgccatacg

SEQ ID NO: 62 - DNA, 2349 bp, Artificial
  psgRNAc BsaI
  gene (219)..(1909): cat CmR chloramphenicol acetyltransferase -  positions are given on the complementary strand : complement (1909-219)
  promoter (220)..(322): cat promoter -  positions are given on the complementary strand : complement (220..322)
  rep_origin (848)..(1393): p15A ori  - positions are given on the complementary strand : complement (848..1393)
  promoter (1510)..(1538): Promoter (BBa_J23119)
  misc_feature (1545)..(1564): Control spacer with 2 BsaI
  misc_RNA (1565)..(1640): gRNA scaffold
  misc_feature (1642)..(1647): part of the tracrRNA
  gene (1648)..(1652): lacI
gaattccggatgagcattcatcaggcgggcaagaatgtgaataaaggccggataaaacttgtgcttatttttctttacggtctttaaaaaggccgtaatatccagctgaacggtctggttataggtacattgagcaactgactgaaatgcctcaaaatgttctttacgatgccattgggatatatcaacggtggtatatccagtgatttttttctccattttagcttccttagctcctgaaaatctcgataactcaaaaaatacgcccggtagtgatcttatttcattatggtgaaagttggaacctcttacgtgccgatcaacgtctcattttcgccaaaagttggcccagggcttcccggtatcaacagggacaccaggatttatttattctgcgaagtgatcttccgtcacaggtatttattcggcgcaaagtgcgtcgggtgatgctgccaacttactgatttagtgtatgatggtgtttttgaggtgctccagtggcttctgtttctatcagctgtccctcctgttcagctactgacggggtggtgcgtaacggcaaaagcaccgccggacatcagcgctagcggagtgtatactggcttactatgttggcactgatgagggtgtcagtgaagtgcttcatgtggcaggagaaaaaaggctgcaccggtgcgtcagcagaatatgtgatacaggatatattccgcttcctcgctcactgactcgctacgctcggtcgttcgactgcggcgagcggaaatggcttacgaacggggcggagatttcctggaagatgccaggaagatacttaacagggaagtgagagggccgcggcaaagccgtttttccataggctccgcccccctgacaagcatcacgaaatctgacgctcaaatcagtggtggcgaaacccgacaggactataaagataccaggcgtttccccctggcggctccctcgtgcgctctcctgttcctgcctttcggtttaccggtgtcattccgctgttatggccgcgtttgtctcattccacgcctgacactcagttccgggtaggcagttcgctccaagctggactgtatgcacgaaccccccgttcagtccgaccgctgcgccttatccggtaactatcgtcttgagtccaacccggaaagacatgcaaaagcaccactggcagcagccactggtaattgatttagaggagttagtcttgaagtcatgcgccggttaaggctaaactgaaaggacaagttttggtgactgcgctcctccaagccagttacctcggttcaaagagttggtagctcagagaaccttcgaaaaaccgccctgcaaggcggttttttcgttttcagagcaagagattacgcgcagaccaaaacgatctcaagaagatcatcttattaatcagataaaatatttctagatttcagtgcaatttatctcttcaaatgtagcacctggctaggaggtgactgaagtatattttaggaattctaaagatctttgacagctagctcagtcctaggtataatactagttgagaccagtctaggtctcggttttagagctagaaatagcaagttaaaataaggctagtccgttatcaacttgaaaaagtggcaccgagtcggtgctttttttggtagtgcagcgcgatcgtaatcaggggggagagcctgagcaaactggcctcaggcatttgagaagcacacggtcacactgcttccggtagtcaataaaccggtaaaccagcaatagacataagcggctatttaacgaccctgccctgaaccgacgaccgggtcgaatttgctttcgaatttctgccattcatccgcttattatcacttattcaggcgtagcaccaggcgtttaagggcaccaataactgccttaaaaaaattacgccccgccctgccactcatcgcagtactgttgtaattcattaagcattctgccgacatggaagccatcacagacggcatgatgaacctgaatcgccagcggcatcagcaccttgtcgccttgcgtataatatttgcccatggtgaaaacgggggcgaagaagttgtccatattggccacgtttaaatcaaaactggtgaaactcacccagggattggctgagacgaaaaacatattctcaataaaccctttagggaaataggccaggttttcaccgtaacacgccacatcttgcgaatatatgtgtagaaactgccggaaatcgtcgtggtattcactccagagcgatgaaaacgtttcagtttgctcatggaaaacggtgtaacaagggtgaacactatcccatatcaccagctcaccgtctttcattgccatacg

SEQ ID NO: 63 - DNA, 9326 bp, Artificial; identical to SEQ ID NO: 60
  pCas9

SEQ ID NO: 64 - DNA, 2433 bp, Artificial
  pCRISPR
ctcgagtccctatcagtgatagagattgacatccctatcagtgatagagatactgagcacatcagcaggacgcactgaccgaattcaactcaacaagtctcagtgtgctgaagttttgggaccattcaaaacagcatagctctaaaacgagacctttgagcttccgagactggtctcagttttgggaccattcaaaacagcatagctctaaaacctcgtagactatttttgtctaaaaaatttcgtaatcgcactatttgtctcagctagacttcagtcttgaaaagcccctgtattactgcatttattaagagtattataccatatttttagttattaagaaataggatcccatggtacgcgtgctagaggcatcaaataaaacgaaaggctcagtcgaaagactgggcctttcgttttatctgttgtttgtcggtgaacgctctcctgagtaggacaaatccgccgccctagacctagggcgttcggctgcggcgagcggtatcagctcactcaaaggcggtaatacggttatccacagaatcaggggataacgcaggaaagaacatgtgagcaaaaggccagcaaaaggccaggaaccgtaaaaaggccgcgttgctggcgtttttccataggctccgcccccctgacgagcatcacaaaaatcgacgctcaagtcagaggtggcgaaacccgacaggactataaagataccaggcgtttccccctggaagctccctcgtgcgctctcctgttccgaccctgccgcttaccggatacctgtccgcctttctcccttcgggaagcgtggcgctttctcaatgctcacgctgtaggtatctcagttcggtgtaggtcgttcgctccaagctgggctgtgtgcacgaaccccccgttcagcccgaccgctgcgccttatccggtaactatcgtcttgagtccaacccggtaagacacgacttatcgccactggcagcagccactggtaacaggattagcagagcgaggtatgtaggcggtgctacagagttcttgaagtggtggcctaactacggctacactagaaggacagtatttggtatctgcgctctgctgaagccagttaccttcggaaaaagagttggtagctcttgatccggcaaacaaaccaccgctggtagcggtggtttttttgtttgcaagcagcagattacgcgcagaaaaaaaggatctcaagaagatcctttgatcttttctacggggtctgacgctcagtggaacgaaaactcacgttaagggattttggtcatgactagtgcttggattctcaccaataaaaaacgcccggcggcaaccgagcgttctgaacaaatccagatggagttctgaggtcattactggatctatcaacaggagtccaagcgagctctcgaaccccagagtcccgctcagaagaactcgtcaagaaggcgatagaaggcgatgcgctgcgaatcgggagcggcgataccgtaaagcacgaggaagcggtcagcccattcgccgccaagctcttcagcaatatcacgggtagccaacgctatgtcctgatagcggtccgccacacccagccggccacagtcgatgaatccagaaaagcggccattttccaccatgatattcggcaagcaggcatcgccatgggtcacgacgagatcctcgccgtcgggcatgcgcgccttgagcctggcgaacagttcggctggcgcgagcccctgatgctcttcgtccagatcatcctgatcgacaagaccggcttccatccgagtacgtgctcgctcgatgcgatgtttcgcttggtggtcgaatgggcaggtagccggatcaagcgtatgcagccgccgcattgcatcagccatgatggatactttctcggcaggagcaaggtgagatgacaggagatcctgccccggcacttcgcccaatagcagccagtcccttcccgcttcagtgacaacgtcgagcacagctgcgcaaggaacgcccgtcgtggccagccacgatagccgcgctgcctcgtcctgcagttcattcagggcaccggacaggtcggtcttgacaaaaagaaccgggcgcccctgcgctgacagccggaacacggcggcatcagagcagccgattgtctgttgtgcccagtcatagccgaatagcctctccacccaagcggccggagaacctgcgtgcaatccatcttgttcaatcatgcgaaacgatcctcatcctgtctcttgatcagatcttgatcccctgcgccatcagatccttggcggcaagaaagccatccagtttactttgcagggcttcccaaccttaccagagggcgccccagctggcaattccgacgtctaagaaaccattattatcatgacattaacctataaaaataggcgtatcacgaggccctttcgtcttcac

SEQ ID NO: 65 - DNA, 2650 bp, Artificial
  pCRRNA
aagatggcagcgcctaaatgtagaatgataaaaggattaagagattaatttccctaaaaatgataaaacaagcgttttgaaagcgcttgtttttttggtttgcagtcagagtagaatagaagtatcaaaaaaagcaccgactcggtgccactttttcaagttgataacggactagccttattttaacttgctatgctgttttgaatggttccaacaagattattttataacttttataacaaataatcaaggagaaattcaaagaaatttatcagccataaaacaatacttaatactcatgaattcaactcaacaagtctcagtgtgctgaagttttgggaccattcaaaacagcatagctctaaaacgagacctttgagcttccgagactggtctcagttttgggaccattcaaaacagcatagctctaaaacctcgtagactatttttgtctaaaaaatttcgtaatcgcactatttgtctcagctagacttcagtcttgaaaagcccctgtattactgcatttattaagagtattataccatatttttagttattaagaaataggatcccatggtacgcgtgctagaggcatcaaataaaacgaaaggctcagtcgaaagactgggcctttcgttttatctgttgtttgtcggtgaacgctctcctgagtaggacaaatccgccgccctagacctagggcgttcggctgcggcgagcggtatcagctcactcaaaggcggtaatacggttatccacagaatcaggggataacgcaggaaagaacatgtgagcaaaaggccagcaaaaggccaggaaccgtaaaaaggccgcgttgctggcgtttttccataggctccgcccccctgacgagcatcacaaaaatcgacgctcaagtcagaggtggcgaaacccgacaggactataaagataccaggcgtttccccctggaagctccctcgtgcgctctcctgttccgaccctgccgcttaccggatacctgtccgcctttctcccttcgggaagcgtggcgctttctcaatgctcacgctgtaggtatctcagttcggtgtaggtcgttcgctccaagctgggctgtgtgcacgaaccccccgttcagcccgaccgctgcgccttatccggtaactatcgtcttgagtccaacccggtaagacacgacttatcgccactggcagcagccactggtaacaggattagcagagcgaggtatgtaggcggtgctacagagttcttgaagtggtggcctaactacggctacactagaaggacagtatttggtatctgcgctctgctgaagccagttaccttcggaaaaagagttggtagctcttgatccggcaaacaaaccaccgctggtagcggtggtttttttgtttgcaagcagcagattacgcgcagaaaaaaaggatctcaagaagatcctttgatcttttctacggggtctgacgctcagtggaacgaaaactcacgttaagggattttggtcatgactagtgcttggattctcaccaataaaaaacgcccggcggcaaccgagcgttctgaacaaatccagatggagttctgaggtcattactggatctatcaacaggagtccaagcgagctctcgaaccccagagtcccgctcagaagaactcgtcaagaaggcgatagaaggcgatgcgctgcgaatcgggagcggcgataccgtaaagcacgaggaagcggtcagcccattcgccgccaagctcttcagcaatatcacgggtagccaacgctatgtcctgatagcggtccgccacacccagccggccacagtcgatgaatccagaaaagcggccattttccaccatgatattcggcaagcaggcatcgccatgggtcacgacgagatcctcgccgtcgggcatgcgcgccttgagcctggcgaacagttcggctggcgcgagcccctgatgctcttcgtccagatcatcctgatcgacaagaccggcttccatccgagtacgtgctcgctcgatgcgatgtttcgcttggtggtcgaatgggcaggtagccggatcaagcgtatgcagccgccgcattgcatcagccatgatggatactttctcggcaggagcaaggtgagatgacaggagatcctgccccggcacttcgcccaatagcagccagtcccttcccgcttcagtgacaacgtcgagcacagctgcgcaaggaacgcccgtcgtggccagccacgatagccgcgctgcctcgtcctgcagttcattcagggcaccggacaggtcggtcttgacaaaaagaaccgggcgcccctgcgctgacagccggaacacggcggcatcagagcagccgattgtctgttgtgcccagtcatagccgaatagcctctccacccaagcggccggagaacctgcgtgcaatccatcttgttcaatcatgcgaaacgatcctcatcctgtctcttgatcagatcttgatcccctgcgccatcagatccttggcggcaagaaagccatccagtttactttgcagggcttcccaaccttaccagagggcgccccagctggcaattccgacgtctaagaaaccattattatcatgacattaacctataaaaataggcgtatcacgaggccctttcgtctt

SEQ ID NO: 66 - DNA, 4085 bp, Artificial
  pLCX
taaaaataggcgtatcacgaggccctttcgtcttcgggcccattaagttctgtctcggcgcgtctgcgtctggctggctggcataaatatctcactcgcaatcaaattcagccgatagcggaacgggaaggcgactggagtgccatgtccggttttcaacaaaccatgcaaatgctgaatgagggcatcgttcccactgcgatgctggttgccaacgatcagatggcgctgggcgcaatgcgcgccattaccgagtccgggctgcgcgttggtgcggatatctcggtagtgggatacgacgataccgaagacagctcatgttatatcccgccgttaaccaccatcaaacaggattttcgcctgctggggcaaaccagcgtggaccgcttgctgcaactctctcagggccaggcggtgaagggcaatcagctgttgcccgtctcactggtgaaaagaaaaaccaccctggcgcccaatacgcaaaccgcctctccccgcgcgttggccgattcattaatgcagctggcacgacaggtttcccgactggaaagcgggcagtgagcgcaacgcaattaatgtgagttagctcactcattaggcaccccaggctttacactttatgcttccggctcgtatgttgtgtggaattgtgagcggataacaatttcacacaggaaacagctatgaccatgattacggattcactggccgtcgttttacaacgtcgtgactgggaaaaccctggcgttacccaacttaatcgccttgcagcacatccccctttcgccagctggcgtaatagcgaagaggcccgcaccgatcgcccttcccaacagttgcgcagcctgaatggcgaatggcgctttgcctggtttccggcaccagaagcggtgccggaaagctggctggagtgcgatcttcctgaggccgatactgtcgtcgtcccctcaaactggcagatgcacggttacgatgcgcccatctacaccaacgtgacctatcccattacggtcaatccgccgtttgttcccacgtagaatccgacgggttgttactcgctcacatttaatgttgatgaaagctggctacaggaaggccagacgcgaattatttttgatggcgttaactcggcgtttcatctgtggtgcaacgggcgctgggtcggttacggccaggacagtcgtttgccgtctgaatttgacctgagcgcatttttacgcgccggagaaaaccgcctcgcggtgatggtgctgcgctggagtgacggcagttatctggaagatcaggatatgtggcggatgagcggcattttccgtgacgtctcgttgctgcataaaccgactacacaaatcagcgatttccatgttgccactcgctttaatgatgatttcagccgcgctgtactggaggctgaagttcagatgtgcggcgagttgcgtgactacctacgggtaacagtttctttatggcagggtgaaacgcaggtcgccagcggcaccgcgcctttcggcggtgaaattatcgatgagcgtggtggttatgccgatcgcgtcacactacgtctgaacgtcgaaaacccgaaactgtggagcgccgaaatcccgaatctctatcgtgcggtggttgaactgcacaccgccgacggcacgctgattgaagcagaagcctgcgatgtcggtttccgcgaggtgcggattgaaaatggtctgctgctgctgaacggcaagccgttgctgattcgaggcgttaaccgtcacgagcatcatcctctgcatggtcaggtcatggatgagcagacgatggtgcaggatatcctgctgatgaagcagaacaactttaacgccgtgcgctgttcgcattatccgaaccatccgctgtggtacacgctgtgcgaccgctacggcctgtatgtggtggatgaagccaatattgaaacccacggcatggtgccaatgaatcgtctgaccgatgatccgcgctggctaccggcgatgagcgaacgcgtaacgcgaatggtgcagcgcgatcgtaatcaggatcccatggtacgcgtgctagaggcatcaaataaaacgaaaggctcagtcgaaagactgggcctttcgttttatctgttgtttgtcggtgaacgctctcctgagtaggacaaatccgccgccctagacctagggcgttcggctgcggcgagcggtatcagctcactcaaaggcggtaatacggttatccacagaatcaggggataacgcaggaaagaacatgtgagcaaaaggccagcaaaaggccaggaaccgtaaaaaggccgcgttgctggcgtttttccataggctccgcccccctgacgagcatcacaaaaatcgacgctcaagtcagaggtggcgaaacccgacaggactataaagataccaggcgtttccccctggaagctccctcgtgcgctctcctgttccgaccctgccgcttaccggatacctgtccgcctttctcccttcgggaagcgtggcgctttctcaatgctcacgctgtaggtatctcagttcggtgtaggtcgttcgctccaagctgggctgtgtgcacgaaccccccgttcagcccgaccgctgcgccttatccggtaactatcgtcttgagtccaacccggtaagacacgacttatcgccactggcagcagccactggtaacaggattagcagagcgaggtatgtaggcggtgctacagagttcttgaagtggtggcctaactacggctacactagaaggacagtatttggtatctgcgctctgctgaagccagttaccttcggaaaaagagttggtagctcttgatccggcaaacaaaccaccgctggtagcggtggtttttttgtttgcaagcagcagattacgcgcagaaaaaaaggatctcaagaagatcctttgatcttttctacggggtctgacgctcagtggaacgaaaactcacgttaagggattttggtcatgactagtgcttggattctcaccaataaaaaacgcccggcggcaaccgagcgttctgaacaaatccagatggagttctgaggtcattactggatctatcaacaggagtccaagcgagctctcgaaccccagagtcccgctcagaagaactcgtcaagaaggcgatagaaggcgatgcgctgcgaatcgggagcggcgataccgtaaagcacgaggaagcggtcagcccattcgccgccaagctcttcagcaatatcacgggtagccaacgctatgtcctgatagcggtccgccacacccagccggccacagtcgatgaatccagaaaagcggccattttccaccatgatattcggcaagcaggcatcgccatgggtcacgacgagatcctcgccgtcgggcatgcgcgccttgagcctggcgaacagttcggctggcgcgagcccctgatgctcttcgtccagatcatcctgatcgacaagaccggcttccatccgagtacgtgctcgctcgatgcgatgtttcgcttggtggtcgaatgggcaggtagccggatcaagcgtatgcagccgccgcattgcatcagccatgatggatactttctcggcaggagcaaggtgagatgacaggagatcctgccccggcacttcgcccaatagcagccagtcccttcccgcttcagtgacaacgtcgagcacagctgcgcaaggaacgcccgtcgtggccagccacgatagccgcgctgcctcgtcctgcagttcattcagggcaccggacaggtcggtcttgacaaaaagaaccgggcgcccctgcgctgacagccggaacacggcggcatcagagcagccgattgtctgttgtgcccagtcatagccgaatagcctctccacccaagcggccggagaacctgcgtgcaatccatcttgttcaatcatgcgaaacgatcctcatcctgtctcttgatcagatcttgatcccctgcgccatcagatccttggcggcaagaaagccatccagtttactttgcagggcttcccaaccttaccagagggcgccccagctggcaattccgacgtctaagaaaccattattatcatgacattaaccta

SEQ ID NO: 67 - DNA, 2349 bp, Artificial; identical to SEQ ID NO: 62
  psgRNAc

SEQ ID NO: 68 - DNA, 8701 bp, Artificial
  pPh1F-Cas9
tcagatccttccgtatttagccagtatgttctctagtgtggttcgttgtttttgcgtgagccatgagaacgaaccattgagatcatacttactttgcatgtcactcaaaaattttgcctcaaaactggtgagctgaatttttgcagttaaagcatcgtgtagtgtttttcttagtccgttacgtaggtaggaatctgatgtaatggttgttggtattttgtcaccattcatttttatctggttgttctcaagttcggttacgagatccatttgtctatctagttcaacttggaaaatcaacgtatcagtcgggcggcctcgcttatcaaccaccaatttcatattgctgtaagtgtttaaatctttacttattggtttcaaaacccattggttaagccttttaaactcatggtagttattttcaagcattaacatgaacttaaattcatcaaggctaatctctatatttgccttgtgagttttcttttgtgttagttcttttaataaccactcataaatcctcatagagtatttgttttcaaaagacttaacatgttccagattatattttatgaatttttttaactggaaaagataaggcaatatctcttcactaaaaactaattctaatttttcgcttgagaacttggcatagtttgtccactggaaaatctcaaagcctttaaccaaaggattcctgatttccacagttctcgtcatcagctctctggttgctttagctaatacaccataagcattttccctactgatgttcatcatctgagcgtattggttataagtgaacgataccgtccgttctttccttgtagggttttcaatcgtggggttgagtagtgccacacagcataaaattagcttggtttcatgctccgttaagtcatagcgactaatcgctagttcatttgctttgaaaacaactaattcagacatacatctcaattggtctaggtgattttaatcactataccaattgagatgggctagtcaatgataattactagtccttttcctttgagttgtgggtatctgtaaattctgctagacctttgctggaaaacttgtaaattctgctagaccctctgtaaattccgctagacctttgtgtgttttttttgtttatattcaagtggttataatttatagaataaagaaagaataaaaaaagataaaaagaatagatcccagccctgtgtataactcactactttagtcagttccgcagtattacaaaaggatgtcgcaaacgctgtttgctcctctacaaaacagaccttaaaaccctaaaggcttaagtagcaccctcgcaagctcggttgcggccgcaatcgggcaaatcgctgaatattccttttgtctccgaccatcaggcacctgagtcgctgtctttttcgtgacattcagttcgctgcgctcacggctctggcagtgaatgggggtaaatggcactacaggcgccttttatggattcatgcaaggaaactacccataatacaagaaaagcccgtcacgggcttctcagggcgttttatggcgggtctgctatgtggtgctatctgactttttgctgttcagcagttcctgccctctgattttccagtctgaccacttcggattatcccgtgacaggtcattcagactggctaatgcacccagtaaggcagcggtatcatcaacggggtctgacgctcagtggaacgaaaactcacgttaagggattttggtcatgagattatcaaaaaggatcttcacctagatccttttaaattaaaaatgaagttttaaatcaatctaaagtatatatgagtaaacttggtctgacagttacgtttccacaaccaattaaccaattctgatttagaaaaactcatcgagcatcaaatgaaactgcaatttattcatatcaggattatcaataccatatttttgaaaaagccgtttctgtaatgaaggagaaaactcaccgaggcagttccataggatggcaagatcctggtatcggtctgcgattccgactcgtccaacatcaatacaacctattaatttcccctcgtcaaaaataaggttatcaagtgagaaatcaccatgagtgacgactgaatccggtgagaatggcaaaagcttatgcatttctttccagacttgttcaacaggccagccattacgctcgtcatcaaaatcactcgcatcaaccaaaccgttattcattcgtgattgcgcctgagcgagacgaaatacgcgatcgctgttaaaaggacaattacaaacaggaatcgaatgcaaccggcgcaggaacactgccagcgcatcaacaatattttcacctgaatcaggatattcttctaatacctggaatgctgttttcccggggatcgcagtggtgagtaaccatgcatcatcaggagtacggataaaatgcttgatggtcggaagaggcataaattccgtcagccagtttagtctgaccatctcatctgtaacatcattggcaacgctacctttgccatgtttcagaaacaactctggcgcatcgggcttcccatacaatcgatagattgtcgcacctgattgcccgacattatcgcgagcccatttatacccatataaatcagcatccatgttggaatttaatcgcggcctcgagcaagacgtttcccgttgaatatggctcataacaccccttgtattactgtttatgtaagcagacagttttattgttcatgatgatatatttttatcttgtgcaatgtaacatcagagattttgagacacaacgtggctttccctgcaggatttcggaggcctgcgttatcccctgattctgtggataaccgtattaccgcctttgagtgagctgataccgctcgccgcagccgaacgccccaaaaagcctcgctttcagcacctgtcgtttcctttcttttcagagggtattttaaataaaaacattaagttatgacgaagaagaacggaaacgccttaaaccggaaaattttcataaatagcgaaaacccgcgaggtcgccgccccgtaacctgtcggatcaccggaaaggacccgtaaagtgataatgattatcatctacatatcacaacgtgcgtggagggactagtggattttacggctagctcagtcctaggtacaatgctagcgaattcattaaagaggagaaaggtacccatggcacgtaccccgagccgtagcagcattggtagcctgcgtagtccgcatacccataaagcaattctgaccagcaccattgaaatcctgaaagaatgtggttatagcggtctgagcattgaaagcgttgcacgtcgtgccggtgcaagcaaaccgaccatttatcgttggtggaccaataaagcagcactgattgccgaagtgtatgaaaatgaaagcgaacaggtgcgtaaatttccggatctgggtagctttaaagccgatctggattttctgctgcgtaatctgtggaaagtttggcgtgaaaccatttgtggtgaagcatttcgttgtgttattgcagaagcacagctggaccctgcaaccctgacccagctgaaagatcagtttatggaacgtcgtcgtgagatgccgaaaaaactggttgaaaatgccattagcaatggtgaactgccgaaagataccaatcgtgaactgctgctggatatgatttttggtttttgttggtatcgcctgctgaccgaacagctgaccgttgaacaggatattgaagaatttaccttcctgctgattaatggtgtttgtccgggtacacagcgttaactagggcccatacccccaattattgaaggccgctaacgcggcctttttttgtttctggtctgcccgacgtacggtgaatctgattcgttaccaattgacatgatacgaaacgtaccgtatcgttaaggttactagagattaaagaggagaaatactagatggataagaaatactcaataggcttagatatcggcacaaatagcgtcggatgggcggtgatcactgatgaatataaggttccgtctaaaaagttcaaggttctgggaaatacagaccgccacagtatcaaaaaaaatcttataggggctcttttatttgacagtggagagacagcggaagcgactcgtctcaaacggacagctcgtagaaggtatacacgtcggaagaatcgtatttgttatctacaggagattttttcaaatgagatggcgaaagtagatgatagtttctttcatcgacttgaagagtcttttttggtggaagaagacaagaagcatgaacgtcatcctatttttggaaatatagtagatgaagttgcttatcatgagaaatatccaactatctatcatctgcgaaaaaaattggtagattctactgataaagcggatttgcgcttaatctatttggccttagcgcatatgattaagtttcgtggtcattttttgattgagggagatttaaatcctgataatagtgatgtggacaaactatttatccagttggtacaaacctacaatcaattatttgaagaaaaccctattaacgcaagtggagtagatgctaaagcgattctttctgcacgattgagtaaatcaagacgattagaaaatctcattgctcagctccccggtgagaagaaaaatggcttatttgggaatctcattgctttgtcattgggtttgacccctaattttaaatcaaattttgatttggcagaagatgctaaattacagctttcaaaagatacttacgatgatgatttagataatttattggcgcaaattggagatcaatatgctgatttgtttttggcagctaagaatttatcagatgctattttactttcagatatcctaagagtaaatactgaaataactaaggctcccctatcagcttcaatgattaaacgctacgatgaacatcatcaagacttgactcttttaaaagctttagttcgacaacaacttccagaaaagtataaagaaatcttttttgatcaatcaaaaaacggatatgcaggttatattgatgggggagctagccaagaagaattttataaatttatcaaaccaattttagaaaaaatggatggtactgaggaattattggtgaaactaaatcgtgaagatttgctgcgcaagcaacggacctttgacaacggctctattccccatcaaattcacttgggtgagctgcatgctattttgagaagacaagaagacttttatccatttttaaaagacaatcgtgagaagattgaaaaaatcttgacttttcgaattccttattatgttggtccattggcgcgtggcaatagtcgttttgcatggatgactcggaagtctgaagaaacaattaccccatggaattttgaagaagttgtcgataaaggtgcttcagctcaatcatttattgaacgcatgacaaactttgataaaaatcttccaaatgaaaaagtactaccaaaacatagtttgctttatgagtattttacggtttataacgaattgacaaaggtcaaatatgttactgaaggaatgcgaaaaccagcatttctttcaggtgaacagaagaaagccattgttgatttactcttcaaaacaaatcgaaaagtaaccgttaagcaattaaaagaagattatttcaaaaaaatagaatgttttgatagtgttgaaatttcaggagttgaagatagatttaatgcttcattaggtacctaccatgatttgctaaaaattattaaagataaagattttttggataatgaagaaaatgaagatatcttagaggatattgttttaacattgaccttatttgaagatagggagatgattgaggaaagacttaaaacatatgctcacctctttgatgataaggtgatgaaacagcttaaacgtcgccgttatactggttggggacgtttgtctcgaaaattgattaatggtattagggataagcaatctggcaaaacaatattagattttttgaaatcagatggttttgccaatcgcaattttatgcagctgatccatgatgatagtttgacatttaaagaagacattcaaaaagcacaagtgtctggacaaggcgatagtttacatgaacatattgcaaatttagctggtagccctgctattaaaaaaggtattttacagactgtaaaagttgttgatgaattggtcaaagtaatggggcggcataagccagaaaatatcgttattgaaatggcacgtgaaaatcagacaactcaaaagggccagaaaaattcgcgagagcgtatgaaacgaatcgaagaaggtatcaaagaattaggaagtcagattcttaaagagcatcctgttgaaaatactcaattgcaaaatgaaaagctctatctctattatctccaaaatggaagagacatgtatgtggaccaagaattagatattaatcgtttaagtgattatgatgtcgatcacattgttccacaaagtttccttaaagacgattcaatagacaataaggtcttaacgcgttctgataaaaatcgtggtaaatcggataacgttccaagtgaagaagtagtcaaaaagatgaaaaactattggagacaacttctaaacgccaagttaatcactcaacgtaagtttgataatttaacgaaagctgaacgtggaggtttgagtgaacttgataaagctggttttatcaaacgccaattggttgaaactcgccaaatcactaagcatgtggcacaaattttggatagtcgcatgaatactaaatacgatgaaaatgataaacttattcgagaggttaaagtgattaccttaaaatctaaattagtttctgacttccgaaaagatttccaattctataaagtacgtgagattaacaattaccatcatgcccatgatgcgtatctaaatgccgtcgttggaactgctttgattaagaaatatccaaaacttgaatcggagtttgtctatggtgattataaagtttatgatgttcgtaaaatgattgctaagtctgagcaagaaataggcaaagcaaccgcaaaatatttcttttactctaatatcatgaacttcttcaaaacagaaattacacttgcaaatggagagattcgcaaacgccctctaatcgaaactaatggggaaactggagaaattgtctgggataaagggcgagattttgccacagtgcgcaaagtattgtccatgccccaagtcaatattgtcaagaaaacagaagtacagacaggcggattctccaaggagtcaattttaccaaaaagaaattcggacaagcttattgctcgtaaaaaagactgggatccaaaaaaatatggtggttttgatagtccaacggtagcttattcagtcctagtggttgctaaggtggaaaaagggaaatcgaagaagttaaaatccgttaaagagttactagggatcacaattatggaaagaagttcctttgaaaaaaatccgattgactttttagaagctaaaggatataaggaagttaaaaaagacttaatcattaaactacctaaatatagtctttttgagttagaaaacggtcgtaaacggatgctggctagtgccggagaattacaaaaaggaaatgagctggctctgccaagcaaatatgtgaattttttatatttagctagtcattatgaaaagttgaagggtagtccagaagataacgaacaaaaacaattgtttgtggagcagcataagcattatttagatgagattattgagcaaatcagtgaattttctaagcgtgttattttagcagatgccaatttagataaagttcttagtgcatataacaaacatagagacaaaccaatacgtgaacaagcagaaaatattattcatttatttacgttgacgaatcttggagctcccgctgcttttaaatattttgatacaacaattgatcgtaaacgatatacgtctacaaaagaagttttagatgccactcttatccatcaatccatcactggtctttatgaaacacgcattgatttgagtcagctaggaggtgactaactcgagtaaggatctccaggcattgcaggcatgcctcgagatgcatggcgcctaacctaaactgatgacgcatcctcacgataatatccgggtaggcgcaatcactttcgtctactccgttacaaagcgaggctgggtatttcccggcctttctgttatccgaaatccactgaaagcacagcggctggctgaggagataaataataaacgaggggctgtatgcacaaagcatcttctgttgagttaagaacgagtatcgagatggcacatagccttgctcaaattggaatcaggtttgtgccaataccagtagaaacagacgaagaatccatgggtatggacagatctcaaaaaaagcaccgactcggtgccactttttcaagttgataacggactagccttattttaacttgctatttctagctctaaaacgggttttcccagtcacgacgtgctagcattatacctaggactgagctagctgtcagccattcgatggtgtcaacgtaaatgcatgccgctcgccttccatgggtatggacagttttccctttgatatgtaacggtgaacagttgttctacttttgtttgttagtcttgatgcttcactgatagatacaagagccataagaacc

SEQ ID NO: 69 - DNA, 4083 bp, Artificial Sequence
  pBAD-MuGam
  misc_feature (2566)..(2595): n is a, c, g, or t
aaaatctcgataactcaaaaaatacgcccggtagtgatcttatttcattatggtgaaagttggaacctcttacgtgccgatcaacgtctcattttcgccaaaagttggcccagggcttcccggtatcaacagggacaccaggatttatttattctgcgaagtgatcttccgtcacaggtatttattcggcgcaaagtgcgtcgggtgatgctgccaacttactgatttagtgtatgatggtgtttttgaggtgctccagtggcttctgtttctatcagctgtccctcctgttcagctactgacggggtggtgcgtaacggcaaaagcaccgccggacatcagcgctagcggagtgtatactggcttactatgttggcactgatgagggtgtcagtgaagtgcttcatgtggcaggagaaaaaaggctgcaccggtgcgtcagcagaatatgtgatacaggatatattccgcttcctcgctcactgactcgctacgctcggtcgttcgactgcggcgagcggaaatggcttacgaacggggcggagatttcctggaagatgccaggaagatacttaacagggaagtgagagggccgcggcaaagccgtttttccataggctccgcccccctgacaagcatcacgaaatctgacgctcaaatcagtggtggcgaaacccgacaggactataaagataccaggcgtttccccctggcggctccctcgtgcgctctcctgttcctgcctttcggtttaccggtgtcattccgctgttatggccgcgtttgtctcattccacgcctgacactcagttccgggtaggcagttcgctccaagctggactgtatgcacgaaccccccgttcagtccgaccgctgcgccttatccggtaactatcgtcttgagtccaacccggaaagacatgcaaaagcaccactggcagcagccactggtaattgatttagaggagttagtcttgaagtcatgcgccggttaaggctaaactgaaaggacaagttttggtgactgcgctcctccaagccagttacctcggttcaaagagttggtagctcagagaaccttcgaaaaaccgccctgcaaggcggttttttcgttttcagagcaagagattacgcgcagaccaaaacgatctcaagaagatcatcttattaatcagataaaatatttctagatttcagtgcaatttatctcttcaaatgtagcacctgaagtcagccccatacgatataagttgtatcgatgcataatgtgcctgtcaaatggacgaagcagggattctgcaaaccctatgctactccgtcaagccgtcaattgtctgattcgttaccaattatgacaacttgacggctacatcattcactttttcttcacaaccggcacggaactcgctcgggctggccccggtgcattttttaaatacccgcgagaaatagagttgatcgtcaaaaccaacattgcgaccgacggtggcgataggcatccgggtggtgctcaaaagcagcttcgcctggctgatacgttggtcctcgcgccagcttaagacgctaatccctaactgctggcggaaaagatgtgacagacgcgacggcgacaagcaaacatgctgtgcgacgctggcgatatcaaaattgctgtctgccaggtgatcgctgatgtactgacaagcctcgcgtacccgattatccatcggtggatggagcgactcgttaatcgcttccatgcgccgcagtaacaattgctcaagcagatttatcgccagcagctccgaatagcgcccttccccttgcccggcgttaatgatttgcccaaacaggtcgctgaaatgcggctggtgcgcttcatccgggcgaaagaaccccgtattggcaaatattgacggccagttaagccattcatgccagtaggcgcgcggacgaaagtaaacccactggtgataccattcgcgagcctccggatgacgaccgtagtgatgaatctctcctggcgggaacagcaaaatatcacccggtcggcaaacaaattctcgtccctgatttttcaccaccccctgaccgcgaatggtgagattgagaatataacctttcattcccagcggtcggtcgataaaaaaatcgagataaccgttggcctcaatcggcgttaaacccgccaccagatgggcattaaacgagtatcccggcagcaggggatcattttgcgcttcagccatacttttcatactcccgccattcagagaagaaaccaattgtccatattgcatcagacattgccgtcactgcgtcttttactggctcttctcgctaaccaaaccggtaaccccgcttattaaaagcattctgtaacaaagcgggaccaaagccatgacaaaaacgcgtaacaaaagtgtctataatcacggcagaaaagtccacattgattatttgcacggcgtcacactttgctatgccatagcatttttatccataagattagcggatcctacctgacgctttttatcgcaactctctactgtttctccatacccgtttttttgggctagcgaattcnnnnnnnnnnnnnnnnnnnnnnnnnnnnnnatggctaaaccagcaaaacgtatcaagagtgccgcagcggcttatgtgccacaaaaccgcgatgcggtgattaccgatattaaacgcatcggggatttacagcgcgaagcatcacgtctggaaacggaaatgaatgatgccatcgcggaaattacggagaaatttgcggcccggattgcaccgattaaaaccgatattgaaaccctttcaaaaggcgttcagggatggtgtgaagcgaaccgcgacgaactgacgaacggcggcaaagtgaagacggcgaatcttgtcaccggtgatgtatcgtggcgggtccgtccaccatcagtaagtattcgtggtatggatgcagtgatggaaacgctggagcgtcttggcctgcaacgctttattcgcacgaagcaggaaatcaacaaggaagcgattttactggaaccgaaagcggtcgcaggcgttgccggaattacagttaaatcaggcattgaggatttttctattattccatttgaacaggaagccggtatttaataattttcccgccctcaaaaaagcaataaagcggctcaatagccgctttattcacatcagcaaaaattatatcgggtagcaccagaagcacacggtcacactgcttccggtagtcaataaaccggtaaaccagcaatagacataagcggctatttaacgaccctgccctgaaccgacgaccgggtcgaatttgctttcgaatttctgccattcatccgcttattatcacttattcaggcgtagcaccaggcgtttaagggcaccaataactgccttaaaaaaattacgccccgccctgccactcatcgcagtactgttgtaattcattaagcattctgccgacatggaagccatcacagacggcatgatgaacctgaatcgccagcggcatcagcaccttgtcgccttgcgtataatatttgcccatggtgaaaacgggggcgaagaagttgtccatattggccacgtttaaatcaaaactggtgaaactcacccagggattggctgagacgaaaaacatattctcaataaaccctttagggaaataggccaggttttcaccgtaacacgccacatcttgcgaatatatgtgtagaaactgccggaaatcgtcgtggtattcactccagagcgatgaaaacgtttcagtttgctcatggaaaacggtgtaacaagggtgaacactatcccatatcaccagctcaccgtctttcattgccatacggaattccggatgagcattcatcaggcgggcaagaatgtgaataaaggccggataaaacttgtgcttatttttctttacggtctttaaaaaggccgtaatatccagctgaacggtctggttataggtacattgagcaactgactgaaatgcctcaaaatgttctttacgatgccattgggatatatcaacggtggtatatccagtgatttttttctccattttagcttccttagctcctg

SEQ ID NO: 70 - DNA, 3979 bp, artificial
  pBAD-LambdaGam
  misc_feature (2570)..(2599): n is a, c, g, or t
aaaatctcgataactcaaaaaatacgcccggtagtgatcttatttcattatggtgaaagttggaacctcttacgtgccgatcaacgtctcattttcgccaaaagttggcccagggcttcccggtatcaacagggacaccaggatttatttattctgcgaagtgatcttccgtcacaggtatttattcggcgcaaagtgcgtcgggtgatgctgccaacttactgatttagtgtatgatggtgtttttgaggtgctccagtggcttctgtttctatcagctgtccctcctgttcagctactgacggggtggtgcgtaacggcaaaagcaccgccggacatcagcgctagcggagtgtatactggcttactatgttggcactgatgagggtgtcagtgaagtgcttcatgtggcaggagaaaaaaggctgcaccggtgcgtcagcagaatatgtgatacaggatatattccgcttcctcgctcactgactcgctacgctcggtcgttcgactgcggcgagcggaaatggcttacgaacggggcggagatttcctggaagatgccaggaagatacttaacagggaagtgagagggccgcggcaaagccgtttttccataggctccgcccccctgacaagcatcacgaaatctgacgctcaaatcagtggtggcgaaacccgacaggactataaagataccaggcgtttccccctggcggctccctcgtgcgctctcctgttcctgcctttcggtttaccggtgtcattccgctgttatggccgcgtttgtctcattccacgcctgacactcagttccgggtaggcagttcgctccaagctggactgtatgcacgaaccccccgttcagtccgaccgctgcgccttatccggtaactatcgtcttgagtccaacccggaaagacatgcaaaagcaccactggcagcagccactggtaattgatttagaggagttagtcttgaagtcatgcgccggttaaggctaaactgaaaggacaagttttggtgactgcgctcctccaagccagttacctcggttcaaagagttggtagctcagagaaccttcgaaaaaccgccctgcaaggcggttttttcgttttcagagcaagagattacgcgcagaccaaaacgatctcaagaagatcatcttattaatcagataaaatatttctagatttcagtgcaatttatctcttcaaatgtagcacctgaagtcagccccatacgatataagttgtatcgatgcataatgtgcctgtcaaatggacgaagcagggattctgcaaaccctatgctactccgtcaagccgtcaattgtctgattcgttaccaattatgacaacttgacggctacatcattcactttttcttcacaaccggcacggaactcgctcgggctggccccggtgcattttttaaatacccgcgagaaatagagttgatcgtcaaaaccaacattgcgaccgacggtggcgataggcatccgggtggtgctcaaaagcagcttcgcctggctgatacgttggtcctcgcgccagcttaagacgctaatccctaactgctggcggaaaagatgtgacagacgcgacggcgacaagcaaacatgctgtgcgacgctggcgatatcaaaattgctgtctgccaggtgatcgctgatgtactgacaagcctcgcgtacccgattatccatcggtggatggagcgactcgttaatcgcttccatgcgccgcagtaacaattgctcaagcagatttatcgccagcagctccgaatagcgcccttccccttgcccggcgttaatgatttgcccaaacaggtcgctgaaatgcggctggtgcgcttcatccgggcgaaagaaccccgtattggcaaatattgacggccagttaagccattcatgccagtaggcgcgcggacgaaagtaaacccactggtgataccattcgcgagcctccggatgacgaccgtagtgatgaatctctcctggcgggaacagcaaaatatcacccggtcggcaaacaaattctcgtccctgatttttcaccaccccctgaccgcgaatggtgagattgagaatataacctttcattcccagcggtcggtcgataaaaaaatcgagataaccgttggcctcaatcggcgttaaacccgccaccagatgggcattaaacgagtatcccggcagcaggggatcattttgcgcttcagccatacttttcatactcccgccattcagagaagaaaccaattgtccatattgcatcagacattgccgtcactgcgtcttttactggctcttctcgctaaccaaaccggtaaccccgcttattaaaagcattctgtaacaaagcgggaccaaagccatgacaaaaacgcgtaacaaaagtgtctataatcacggcagaaaagtccacattgattatttgcacggcgtcacactttgctatgccatagcatttttatccataagattagcggatcctacctgacgctttttatcgcaactctctactgtttctccatacccgtttttttgggctagcgaattcgagcnnnnnnnnnnnnnnnnnnnnnnnnnnnnnnatggatattaatactgaaactgagatcaagcaaaagcattcactaaccccctttcctgttttcctaatcagcccggcatttcgcgggcgatattttcacagctatttcaggagttcagccatgaacgcttattacattcaggatcgtcttgaggctcagagctgggcgcgtcactaccagcagctcgcccgtgaagagaaagaggcagaactggcagacgacatggaaaaaggcctgccccagcacctgtttgaatcgctatgcatcgatcatttgcaacgccacggggccagcaaaaaatccattacccgtgcgtttgatgacgatgttgagtttcaggagcgcatggcagaacacatccggtacatggttgaaaccattgctcaccaccaggttgatattgattcagaggtataataattttcccgccctcaaaaaagcaataaagcggctcaatagccgctttattcacatcagcaaaaattatatcgggtagcaccagaagcacacggtcacactgcttccggtagtcaataaaccggtaaaccagcaatagacataagcggctatttaacgaccctgccctgaaccgacgaccgggtcgaatttgctttcgaatttctgccattcatccgcttattatcacttattcaggcgtagcaccaggcgtttaagggcaccaataactgccttaaaaaaattacgccccgccctgccactcatcgcagtactgttgtaattcattaagcattctgccgacatggaagccatcacagacggcatgatgaacctgaatcgccagcggcatcagcaccttgtcgccttgcgtataatatttgcccatggtgaaaacgggggcgaagaagttgtccatattggccacgtttaaatcaaaactggtgaaactcacccagggattggctgagacgaaaaacatattctcaataaaccctttagggaaataggccaggttttcaccgtaacacgccacatcttgcgaatatatgtgtagaaactgccggaaatcgtcgtggtattcactccagagcgatgaaaacgtttcagtttgctcatggaaaacggtgtaacaagggtgaacactatcccatatcaccagctcaccgtctttcattgccatacggaattccggatgagcattcatcaggcgggcaagaatgtgaataaaggccggataaaacttgtgcttatttttctttacggtctttaaaaaggccgtaatatccagctgaacggtctggttataggtacattgagcaactgactgaaatgcctcaaaatgttctttacgatgccattgggatatatcaacggtggtatatccagtgatttttttctccattttagcttccttagctcctg

SEQ ID NO: 71 - DNA, 10701 bp, Artificial
  pCas9-MuGam
  misc_feature (9946)..(9976): n is a, c, g, or t
tcagatccttccgtatttagccagtatgttctctagtgtggttcgttgtttttgcgtgagccatgagaacgaaccattgagatcatacttactttgcatgtcactcaaaaattttgcctcaaaactggtgagctgaatttttgcagttaaagcatcgtgtagtgtttttcttagtccgttacgtaggtaggaatctgatgtaatggttgttggtattttgtcaccattcatttttatctggttgttctcaagttcggttacgagatccatttgtctatctagttcaacttggaaaatcaacgtatcagtcgggcggcctcgcttatcaaccaccaatttcatattgctgtaagtgtttaaatctttacttattggtttcaaaacccattggttaagccttttaaactcatggtagttattttcaagcattaacatgaacttaaattcatcaaggctaatctctatatttgccttgtgagttttcttttgtgttagttcttttaataaccactcataaatcctcatagagtatttgttttcaaaagacttaacatgttccagattatattttatgaatttttttaactggaaaagataaggcaatatctcttcactaaaaactaattctaatttttcgcttgagaacttggcatagtttgtccactggaaaatctcaaagcctttaaccaaaggattcctgatttccacagttctcgtcatcagctctctggttgctttagctaatacaccataagcattttccctactgatgttcatcatctgagcgtattggttataagtgaacgataccgtccgttctttccttgtagggttttcaatcgtggggttgagtagtgccacacagcataaaattagcttggtttcatgctccgttaagtcatagcgactaatcgctagttcatttgctttgaaaacaactaattcagacatacatctcaattggtctaggtgattttaatcactataccaattgagatgggctagtcaatgataattactagtccttttcctttgagttgtgggtatctgtaaattctgctagacctttgctggaaaacttgtaaattctgctagaccctctgtaaattccgctagacctttgtgtgttttttttgtttatattcaagtggttataatttatagaataaagaaagaataaaaaaagataaaaagaatagatcccagccctgtgtataactcactactttagtcagttccgcagtattacaaaaggatgtcgcaaacgctgtttgctcctctacaaaacagaccttaaaaccctaaaggcttaagtagcaccctcgcaagctcggttgcggccgcaatcgggcaaatcgctgaatattccttttgtctccgaccatcaggcacctgagtcgctgtctttttcgtgacattcagttcgctgcgctcacggctctggcagtgaatgggggtaaatggcactacaggcgccttttatggattcatgcaaggaaactacccataatacaagaaaagcccgtcacgggcttctcagggcgttttatggcgggtctgctatgtggtgctatctgactttttgctgttcagcagttcctgccctctgattttccagtctgaccacttcggattatcccgtgacaggtcattcagactggctaatgcacccagtaaggcagcggtatcatcaacggggtctgacgctcagtggaacgaaaactcacgttaagggattttggtcatgagattatcaaaaaggatcttcacctagatccttttaaattaaaaatgaagttttaaatcaatctaaagtatatatgagtaaacttggtctgacagttacgtttccacaaccaattaaccaattctgatttagaaaaactcatcgagcatcaaatgaaactgcaatttattcatatcaggattatcaataccatatttttgaaaaagccgtttctgtaatgaaggagaaaactcaccgaggcagttccataggatggcaagatcctggtatcggtctgcgattccgactcgtccaacatcaatacaacctattaatttcccctcgtcaaaaataaggttatcaagtgagaaatcaccatgagtgacgactgaatccggtgagaatggcaaaagcttatgcatttctttccagacttgttcaacaggccagccattacgctcgtcatcaaaatcactcgcatcaaccaaaccgttattcattcgtgattgcgcctgagcgagacgaaatacgcgatcgctgttaaaaggacaattacaaacaggaatcgaatgcaaccggcgcaggaacactgccagcgcatcaacaatattttcacctgaatcaggatattcttctaatacctggaatgctgttttcccggggatcgcagtggtgagtaaccatgcatcatcaggagtacggataaaatgcttgatggtcggaagaggcataaattccgtcagccagtttagtctgaccatctcatctgtaacatcattggcaacgctacctttgccatgtttcagaaacaactctggcgcatcgggcttcccatacaatcgatagattgtcgcacctgattgcccgacattatcgcgagcccatttatacccatataaatcagcatccatgttggaatttaatcgcggcctcgagcaagacgtttcccgttgaatatggctcataacaccccttgtattactgtttatgtaagcagacagttttattgttcatgatgatatatttttatcttgtgcaatgtaacatcagagattttgagacacaacgtggctttccctgcaggatttcggaggcctgcgttatcccctgattctgtggataaccgtattaccgcctttgagtgagctgataccgctcgccgcagccgaacgccccaaaaagcctcgctttcagcacctgtcgtttcctttcttttcagagggtattttaaataaaaacattaagttatgacgaagaagaacggaaacgccttaaaccggaaaattttcataaatagcgaaaacccgcgaggtcgccgccccgtaacctgtcggatcaccggaaaggacccgtaaagtgataatgattatcatctacatatcacaacgtgcgtggagggactagtggattttacggctagctcagtcctaggtacaatgctagcgaattcattaaagaggagaaaggtacccatggcacgtaccccgagccgtagcagcattggtagcctgcgtagtccgcatacccataaagcaattctgaccagcaccattgaaatcctgaaagaatgtggttatagcggtctgagcattgaaagcgttgcacgtcgtgccggtgcaagcaaaccgaccatttatcgttggtggaccaataaagcagcactgattgccgaagtgtatgaaaatgaaagcgaacaggtgcgtaaatttccggatctgggtagctttaaagccgatctggattttctgctgcgtaatctgtggaaagtttggcgtgaaaccatttgtggtgaagcatttcgttgtgttattgcagaagcacagctggaccctgcaaccctgacccagctgaaagatcagtttatggaacgtcgtcgtgagatgccgaaaaaactggttgaaaatgccattagcaatggtgaactgccgaaagataccaatcgtgaactgctgctggatatgatttttggtttttgttggtatcgcctgctgaccgaacagctgaccgttgaacaggatattgaagaatttaccttcctgctgattaatggtgtttgtccgggtacacagcgttaactagggcccatacccccaattattgaaggccgctaacgcggcctttttttgtttctggtctgcccgacgtacggtgaatctgattcgttaccaattgacatgatacgaaacgtaccgtatcgttaaggttactagagattaaagaggagaaatactagatggataagaaatactcaataggcttagatatcggcacaaatagcgtcggatgggcggtgatcactgatgaatataaggttccgtctaaaaagttcaaggttctgggaaatacagaccgccacagtatcaaaaaaaatcttataggggctcttttatttgacagtggagagacagcggaagcgactcgtctcaaacggacagctcgtagaaggtatacacgtcggaagaatcgtatttgttatctacaggagattttttcaaatgagatggcgaaagtagatgatagtttctttcatcgacttgaagagtcttttttggtggaagaagacaagaagcatgaacgtcatcctatttttggaaatatagtagatgaagttgcttatcatgagaaatatccaactatctatcatctgcgaaaaaaattggtagattctactgataaagcggatttgcgcttaatctatttggccttagcgcatatgattaagtttcgtggtcattttttgattgagggagatttaaatcctgataatagtgatgtggacaaactatttatccagttggtacaaacctacaatcaattatttgaagaaaaccctattaacgcaagtggagtagatgctaaagcgattctttctgcacgattgagtaaatcaagacgattagaaaatctcattgctcagctccccggtgagaagaaaaatggcttatttgggaatctcattgctttgtcattgggtttgacccctaattttaaatcaaattttgatttggcagaagatgctaaattacagctttcaaaagatacttacgatgatgatttagataatttattggcgcaaattggagatcaatatgctgatttgtttttggcagctaagaatttatcagatgctattttactttcagatatcctaagagtaaatactgaaataactaaggctcccctatcagcttcaatgattaaacgctacgatgaacatcatcaagacttgactcttttaaaagctttagttcgacaacaacttccagaaaagtataaagaaatcttttttgatcaatcaaaaaacggatatgcaggttatattgatgggggagctagccaagaagaattttataaatttatcaaaccaattttagaaaaaatggatggtactgaggaattattggtgaaactaaatcgtgaagatttgctgcgcaagcaacggacctttgacaacggctctattccccatcaaattcacttgggtgagctgcatgctattttgagaagacaagaagacttttatccatttttaaaagacaatcgtgagaagattgaaaaaatcttgacttttcgaattccttattatgttggtccattggcgcgtggcaatagtcgttttgcatggatgactcggaagtctgaagaaacaattaccccatggaattttgaagaagttgtcgataaaggtgcttcagctcaatcatttattgaacgcatgacaaactttgataaaaatcttccaaatgaaaaagtactaccaaaacatagtttgctttatgagtattttacggtttataacgaattgacaaaggtcaaatatgttactgaaggaatgcgaaaaccagcatttctttcaggtgaacagaagaaagccattgttgatttactcttcaaaacaaatcgaaaagtaaccgttaagcaattaaaagaagattatttcaaaaaaatagaatgttttgatagtgttgaaatttcaggagttgaagatagatttaatgcttcattaggtacctaccatgatttgctaaaaattattaaagataaagattttttggataatgaagaaaatgaagatatcttagaggatattgttttaacattgaccttatttgaagatagggagatgattgaggaaagacttaaaacatatgctcacctctttgatgataaggtgatgaaacagcttaaacgtcgccgttatactggttggggacgtttgtctcgaaaattgattaatggtattagggataagcaatctggcaaaacaatattagattttttgaaatcagatggttttgccaatcgcaattttatgcagctgatccatgatgatagtttgacatttaaagaagacattcaaaaagcacaagtgtctggacaaggcgatagtttacatgaacatattgcaaatttagctggtagccctgctattaaaaaaggtattttacagactgtaaaagttgttgatgaattggtcaaagtaatggggcggcataagccagaaaatatcgttattgaaatggcacgtgaaaatcagacaactcaaaagggccagaaaaattcgcgagagcgtatgaaacgaatcgaagaaggtatcaaagaattaggaagtcagattcttaaagagcatcctgttgaaaatactcaattgcaaaatgaaaagctctatctctattatctccaaaatggaagagacatgtatgtggaccaagaattagatattaatcgtttaagtgattatgatgtcgatcacattgttccacaaagtttccttaaagacgattcaatagacaataaggtcttaacgcgttctgataaaaatcgtggtaaatcggataacgttccaagtgaagaagtagtcaaaaagatgaaaaactattggagacaacttctaaacgccaagttaatcactcaacgtaagtttgataatttaacgaaagctgaacgtggaggtttgagtgaacttgataaagctggttttatcaaacgccaattggttgaaactcgccaaatcactaagcatgtggcacaaattttggatagtcgcatgaatactaaatacgatgaaaatgataaacttattcgagaggttaaagtgattaccttaaaatctaaattagtttctgacttccgaaaagatttccaattctataaagtacgtgagattaacaattaccatcatgcccatgatgcgtatctaaatgccgtcgttggaactgctttgattaagaaatatccaaaacttgaatcggagtttgtctatggtgattataaagtttatgatgttcgtaaaatgattgctaagtctgagcaagaaataggcaaagcaaccgcaaaatatttcttttactctaatatcatgaacttcttcaaaacagaaattacacttgcaaatggagagattcgcaaacgccctctaatcgaaactaatggggaaactggagaaattgtctgggataaagggcgagattttgccacagtgcgcaaagtattgtccatgccccaagtcaatattgtcaagaaaacagaagtacagacaggcggattctccaaggagtcaattttaccaaaaagaaattcggacaagcttattgctcgtaaaaaagactgggatccaaaaaaatatggtggttttgatagtccaacggtagcttattcagtcctagtggttgctaaggtggaaaaagggaaatcgaagaagttaaaatccgttaaagagttactagggatcacaattatggaaagaagttcctttgaaaaaaatccgattgactttttagaagctaaaggatataaggaagttaaaaaagacttaatcattaaactacctaaatatagtctttttgagttagaaaacggtcgtaaacggatgctggctagtgccggagaattacaaaaaggaaatgagctggctctgccaagcaaatatgtgaattttttatatttagctagtcattatgaaaagttgaagggtagtccagaagataacgaacaaaaacaattgtttgtggagcagcataagcattatttagatgagattattgagcaaatcagtgaattttctaagcgtgttattttagcagatgccaatttagataaagttcttagtgcatataacaaacatagagacaaaccaatacgtgaacaagcagaaaatattattcatttatttacgttgacgaatcttggagctcccgctgcttttaaatattttgatacaacaattgatcgtaaacgatatacgtctacaaaagaagttttagatgccactcttatccatcaatccatcactggtctttatgaaacacgcattgatttgagtcagctaggaggtgactaactcgagtaaggatctccaggcattgcaggcatgcctcgagatgcatggcgcctaacctaaactgatgacgcatcctcacgataatatccgggtaggcgcaatcactttcgtctactccgttacaaagcgaggctgggtatttcccggcctttctgttatccgaaatccactgaaagcacagcggctggctgaggagataaataataaacgaggggctgtatgcacaaagcatcttctgttgagttaagaacgagtatcgagatggcacatagccttgctcaaattggaatcaggtttgtgccaataccagtagaaacagacgaagaatccatgggtatggacagatctcaaaaaaagcaccgactcggtgccactttttcaagttgataacggactagccttattttaacttgctatttctagctctaaaacgggttttcccagtcacgacgtgctagcattatacctaggactgagctagctgtcagccattcgatggtgtcaacgtaaatgcatgccgcttcgcctcgtccggcgtagaggatctgctcatgtttgacagcttatcatcgatgcataatgtgcctgtcaaatggacgaagcagggattctgcaaaccctatgctactccgtcaagccgtcaattgtctgattcgttaccaattatgacaacttgacggctacatcattcactttttcttcacaaccggcacggaactcgctcgggctggccccggtgcattttttaaatacccgcgagaaatagagttgatcgtcaaaaccaacattgcgaccgacggtggcgataggcatccgggtggtgctcaaaagcagcttcgcctggctgatacgttggtcctcgcgccagcttaagacgctaatccctaactgctggcggaaaagatgtgacagacgcgacggcgacaagcaaacatgctgtgcgacgctggcgatatcaaaattgctgtctgccaggtgatcgctgatgtactgacaagcctcgcgtacccgattatccatcggtggatggagcgactcgttaatcgcttccatgcgccgcagtaacaattgctcaagcagatttatcgccagcagctccgaatagcgcccttccccttgcccggcgttaatgatttgcccaaacaggtcgctgaaatgcggctggtgcgcttcatccgggcgaaagaaccccgtattggcaaatattgacggccagttaagccattcatgccagtaggcgcgcggacgaaagtaaacccactggtgataccattcgcgagcctccggatgacgaccgtagtgatgaatctctcctggcgggaacagcaaaatatcacccggtcggcaaacaaattctcgtccctgatttttcaccaccccctgaccgcgaatggtgagattgagaatataacctttcattcccagcggtcggtcgataaaaaaatcgagataaccgttggcctcaatcggcgttaaacccgccaccagatgggcattaaacgagtatcccggcagcaggggatcattttgcgcttcagccatacttttcatactcccgccattcagagaagaaaccaattgtccatattgcatcagacattgccgtcactgcgtcttttactggctcttctcgctaaccaaaccggtaaccccgcttattaaaagcattctgtaacaaagcgggaccaaagccatgacaaaaacgcgtaacaaaagtgtctataatcacggcagaaaagtccacattgattatttgcacggcgtcacactttgctatgccatagcatttttatccataagattagcggatcctacctgacgctttttatcgcaactctctactgtttctccatacccgtttttttgggctagcgaattcnnnnnnnnnnnnnnnnnnnnnnnnnnnnnnnatggctaaaccagcaaaacgtatcaagagtgccgcagcggcttatgtgccacaaaaccgcgatgcggtgattaccgatattaaacgcatcggggatttacagcgcgaagcatcacgtctggaaacggaaatgaatgatgccatcgcggaaattacggagaaatttgcggcccggattgcaccgattaaaaccgatattgaaaccctttcaaaaggcgttcagggatggtgtgaagcgaaccgcgacgaactgacgaacggcggcaaagtgaagacggcgaatcttgtcaccggtgatgtatcgtggcgggtccgtccaccatcagtaagtattcgtggtatggatgcagtgatggaaacgctggagcgtcttggcctgcaacgctttattcgcacgaagcaggaaatcaacaaggaagcgattttactggaaccgaaagcggtcgcaggcgttgccggaattacagttaaatcaggcattgaggatttttctattattccatttgaacaggaagccggtatttaattggctgttttggcggatgagagaagattttcagcggaaacacagaaaaaagcccgcacctgacagtgcgggctttttttttcgaccaaaggtccatgggtatggacagttttccctttgatatgtaacggtgaacagttgttctacttttgtttgttagtcttgatgcttcactgatagatacaagagccataagaacc

SEQ ID NO: 72 - DNA, 10593 bp, Artificial
  pCas9-LambdaGam
  misc_feature (9946)..(9976): n is a, c, g, or t
tcagatccttccgtatttagccagtatgttctctagtgtggttcgttgtttttgcgtgagccatgagaacgaaccattgagatcatacttactttgcatgtcactcaaaaattttgcctcaaaactggtgagctgaatttttgcagttaaagcatcgtgtagtgtttttcttagtccgttacgtaggtaggaatctgatgtaatggttgttggtattttgtcaccattcatttttatctggttgttctcaagttcggttacgagatccatttgtctatctagttcaacttggaaaatcaacgtatcagtcgggcggcctcgcttatcaaccaccaatttcatattgctgtaagtgtttaaatctttacttattggtttcaaaacccattggttaagccttttaaactcatggtagttattttcaagcattaacatgaacttaaattcatcaaggctaatctctatatttgccttgtgagttttcttttgtgttagttcttttaataaccactcataaatcctcatagagtatttgttttcaaaagacttaacatgttccagattatattttatgaatttttttaactggaaaagataaggcaatatctcttcactaaaaactaattctaatttttcgcttgagaacttggcatagtttgtccactggaaaatctcaaagcctttaaccaaaggattcctgatttccacagttctcgtcatcagctctctggttgctttagctaatacaccataagcattttccctactgatgttcatcatctgagcgtattggttataagtgaacgataccgtccgttctttccttgtagggttttcaatcgtggggttgagtagtgccacacagcataaaattagcttggtttcatgctccgttaagtcatagcgactaatcgctagttcatttgctttgaaaacaactaattcagacatacatctcaattggtctaggtgattttaatcactataccaattgagatgggctagtcaatgataattactagtccttttcctttgagttgtgggtatctgtaaattctgctagacctttgctggaaaacttgtaaattctgctagaccctctgtaaattccgctagacctttgtgtgttttttttgtttatattcaagtggttataatttatagaataaagaaagaataaaaaaagataaaaagaatagatcccagccctgtgtataactcactactttagtcagttccgcagtattacaaaaggatgtcgcaaacgctgtttgctcctctacaaaacagaccttaaaaccctaaaggcttaagtagcaccctcgcaagctcggttgcggccgcaatcgggcaaatcgctgaatattccttttgtctccgaccatcaggcacctgagtcgctgtctttttcgtgacattcagttcgctgcgctcacggctctggcagtgaatgggggtaaatggcactacaggcgccttttatggattcatgcaaggaaactacccataatacaagaaaagcccgtcacgggcttctcagggcgttttatggcgggtctgctatgtggtgctatctgactttttgctgttcagcagttcctgccctctgattttccagtctgaccacttcggattatcccgtgacaggtcattcagactggctaatgcacccagtaaggcagcggtatcatcaacggggtctgacgctcagtggaacgaaaactcacgttaagggattttggtcatgagattatcaaaaaggatcttcacctagatccttttaaattaaaaatgaagttttaaatcaatctaaagtatatatgagtaaacttggtctgacagttacgtttccacaaccaattaaccaattctgatttagaaaaactcatcgagcatcaaatgaaactgcaatttattcatatcaggattatcaataccatatttttgaaaaagccgtttctgtaatgaaggagaaaactcaccgaggcagttccataggatggcaagatcctggtatcggtctgcgattccgactcgtccaacatcaatacaacctattaatttcccctcgtcaaaaataaggttatcaagtgagaaatcaccatgagtgacgactgaatccggtgagaatggcaaaagcttatgcatttctttccagacttgttcaacaggccagccattacgctcgtcatcaaaatcactcgcatcaaccaaaccgttattcattcgtgattgcgcctgagcgagacgaaatacgcgatcgctgttaaaaggacaattacaaacaggaatcgaatgcaaccggcgcaggaacactgccagcgcatcaacaatattttcacctgaatcaggatattcttctaatacctggaatgctgttttcccggggatcgcagtggtgagtaaccatgcatcatcaggagtacggataaaatgcttgatggtcggaagaggcataaattccgtcagccagtttagtctgaccatctcatctgtaacatcattggcaacgctacctttgccatgtttcagaaacaactctggcgcatcgggcttcccatacaatcgatagattgtcgcacctgattgcccgacattatcgcgagcccatttatacccatataaatcagcatccatgttggaatttaatcgcggcctcgagcaagacgtttcccgttgaatatggctcataacaccccttgtattactgtttatgtaagcagacagttttattgttcatgatgatatatttttatcttgtgcaatgtaacatcagagattttgagacacaacgtggctttccctgcaggatttcggaggcctgcgttatcccctgattctgtggataaccgtattaccgcctttgagtgagctgataccgctcgccgcagccgaacgccccaaaaagcctcgctttcagcacctgtcgtttcctttcttttcagagggtattttaaataaaaacattaagttatgacgaagaagaacggaaacgccttaaaccggaaaattttcataaatagcgaaaacccgcgaggtcgccgccccgtaacctgtcggatcaccggaaaggacccgtaaagtgataatgattatcatctacatatcacaacgtgcgtggagggactagtggattttacggctagctcagtcctaggtacaatgctagcgaattcattaaagaggagaaaggtacccatggcacgtaccccgagccgtagcagcattggtagcctgcgtagtccgcatacccataaagcaattctgaccagcaccattgaaatcctgaaagaatgtggttatagcggtctgagcattgaaagcgttgcacgtcgtgccggtgcaagcaaaccgaccatttatcgttggtggaccaataaagcagcactgattgccgaagtgtatgaaaatgaaagcgaacaggtgcgtaaatttccggatctgggtagctttaaagccgatctggattttctgctgcgtaatctgtggaaagtttggcgtgaaaccatttgtggtgaagcatttcgttgtgttattgcagaagcacagctggaccctgcaaccctgacccagctgaaagatcagtttatggaacgtcgtcgtgagatgccgaaaaaactggttgaaaatgccattagcaatggtgaactgccgaaagataccaatcgtgaactgctgctggatatgatttttggtttttgttggtatcgcctgctgaccgaacagctgaccgttgaacaggatattgaagaatttaccttcctgctgattaatggtgtttgtccgggtacacagcgttaactagggcccatacccccaattattgaaggccgctaacgcggcctttttttgtttctggtctgcccgacgtacggtgaatctgattcgttaccaattgacatgatacgaaacgtaccgtatcgttaaggttactagagattaaagaggagaaatactagatggataagaaatactcaataggcttagatatcggcacaaatagcgtcggatgggcggtgatcactgatgaatataaggttccgtctaaaaagttcaaggttctgggaaatacagaccgccacagtatcaaaaaaaatcttataggggctcttttatttgacagtggagagacagcggaagcgactcgtctcaaacggacagctcgtagaaggtatacacgtcggaagaatcgtatttgttatctacaggagattttttcaaatgagatggcgaaagtagatgatagtttctttcatcgacttgaagagtcttttttggtggaagaagacaagaagcatgaacgtcatcctatttttggaaatatagtagatgaagttgcttatcatgagaaatatccaactatctatcatctgcgaaaaaaattggtagattctactgataaagcggatttgcgcttaatctatttggccttagcgcatatgattaagtttcgtggtcattttttgattgagggagatttaaatcctgataatagtgatgtggacaaactatttatccagttggtacaaacctacaatcaattatttgaagaaaaccctattaacgcaagtggagtagatgctaaagcgattctttctgcacgattgagtaaatcaagacgattagaaaatctcattgctcagctccccggtgagaagaaaaatggcttatttgggaatctcattgctttgtcattgggtttgacccctaattttaaatcaaattttgatttggcagaagatgctaaattacagctttcaaaagatacttacgatgatgatttagataatttattggcgcaaattggagatcaatatgctgatttgtttttggcagctaagaatttatcagatgctattttactttcagatatcctaagagtaaatactgaaataactaaggctcccctatcagcttcaatgattaaacgctacgatgaacatcatcaagacttgactcttttaaaagctttagttcgacaacaacttccagaaaagtataaagaaatcttttttgatcaatcaaaaaacggatatgcaggttatattgatgggggagctagccaagaagaattttataaatttatcaaaccaattttagaaaaaatggatggtactgaggaattattggtgaaactaaatcgtgaagatttgctgcgcaagcaacggacctttgacaacggctctattccccatcaaattcacttgggtgagctgcatgctattttgagaagacaagaagacttttatccatttttaaaagacaatcgtgagaagattgaaaaaatcttgacttttcgaattccttattatgttggtccattggcgcgtggcaatagtcgttttgcatggatgactcggaagtctgaagaaacaattaccccatggaattttgaagaagttgtcgataaaggtgcttcagctcaatcatttattgaacgcatgacaaactttgataaaaatcttccaaatgaaaaagtactaccaaaacatagtttgctttatgagtattttacggtttataacgaattgacaaaggtcaaatatgttactgaaggaatgcgaaaaccagcatttctttcaggtgaacagaagaaagccattgttgatttactcttcaaaacaaatcgaaaagtaaccgttaagcaattaaaagaagattatttcaaaaaaatagaatgttttgatagtgttgaaatttcaggagttgaagatagatttaatgcttcattaggtacctaccatgatttgctaaaaattattaaagataaagattttttggataatgaagaaaatgaagatatcttagaggatattgttttaacattgaccttatttgaagatagggagatgattgaggaaagacttaaaacatatgctcacctctttgatgataaggtgatgaaacagcttaaacgtcgccgttatactggttggggacgtttgtctcgaaaattgattaatggtattagggataagcaatctggcaaaacaatattagattttttgaaatcagatggttttgccaatcgcaattttatgcagctgatccatgatgatagtttgacatttaaagaagacattcaaaaagcacaagtgtctggacaaggcgatagtttacatgaacatattgcaaatttagctggtagccctgctattaaaaaaggtattttacagactgtaaaagttgttgatgaattggtcaaagtaatggggcggcataagccagaaaatatcgttattgaaatggcacgtgaaaatcagacaactcaaaagggccagaaaaattcgcgagagcgtatgaaacgaatcgaagaaggtatcaaagaattaggaagtcagattcttaaagagcatcctgttgaaaatactcaattgcaaaatgaaaagctctatctctattatctccaaaatggaagagacatgtatgtggaccaagaattagatattaatcgtttaagtgattatgatgtcgatcacattgttccacaaagtttccttaaagacgattcaatagacaataaggtcttaacgcgttctgataaaaatcgtggtaaatcggataacgttccaagtgaagaagtagtcaaaaagatgaaaaactattggagacaacttctaaacgccaagttaatcactcaacgtaagtttgataatttaacgaaagctgaacgtggaggtttgagtgaacttgataaagctggttttatcaaacgccaattggttgaaactcgccaaatcactaagcatgtggcacaaattttggatagtcgcatgaatactaaatacgatgaaaatgataaacttattcgagaggttaaagtgattaccttaaaatctaaattagtttctgacttccgaaaagatttccaattctataaagtacgtgagattaacaattaccatcatgcccatgatgcgtatctaaatgccgtcgttggaactgctttgattaagaaatatccaaaacttgaatcggagtttgtctatggtgattataaagtttatgatgttcgtaaaatgattgctaagtctgagcaagaaataggcaaagcaaccgcaaaatatttcttttactctaatatcatgaacttcttcaaaacagaaattacacttgcaaatggagagattcgcaaacgccctctaatcgaaactaatggggaaactggagaaattgtctgggataaagggcgagattttgccacagtgcgcaaagtattgtccatgccccaagtcaatattgtcaagaaaacagaagtacagacaggcggattctccaaggagtcaattttaccaaaaagaaattcggacaagcttattgctcgtaaaaaagactgggatccaaaaaaatatggtggttttgatagtccaacggtagcttattcagtcctagtggttgctaaggtggaaaaagggaaatcgaagaagttaaaatccgttaaagagttactagggatcacaattatggaaagaagttcctttgaaaaaaatccgattgactttttagaagctaaaggatataaggaagttaaaaaagacttaatcattaaactacctaaatatagtctttttgagttagaaaacggtcgtaaacggatgctggctagtgccggagaattacaaaaaggaaatgagctggctctgccaagcaaatatgtgaattttttatatttagctagtcattatgaaaagttgaagggtagtccagaagataacgaacaaaaacaattgtttgtggagcagcataagcattatttagatgagattattgagcaaatcagtgaattttctaagcgtgttattttagcagatgccaatttagataaagttcttagtgcatataacaaacatagagacaaaccaatacgtgaacaagcagaaaatattattcatttatttacgttgacgaatcttggagctcccgctgcttttaaatattttgatacaacaattgatcgtaaacgatatacgtctacaaaagaagttttagatgccactcttatccatcaatccatcactggtctttatgaaacacgcattgatttgagtcagctaggaggtgactaactcgagtaaggatctccaggcattgcaggcatgcctcgagatgcatggcgcctaacctaaactgatgacgcatcctcacgataatatccgggtaggcgcaatcactttcgtctactccgttacaaagcgaggctgggtatttcccggcctttctgttatccgaaatccactgaaagcacagcggctggctgaggagataaataataaacgaggggctgtatgcacaaagcatcttctgttgagttaagaacgagtatcgagatggcacatagccttgctcaaattggaatcaggtttgtgccaataccagtagaaacagacgaagaatccatgggtatggacagatctcaaaaaaagcaccgactcggtgccactttttcaagttgataacggactagccttattttaacttgctatttctagctctaaaacgggttttcccagtcacgacgtgctagcattatacctaggactgagctagctgtcagccattcgatggtgtcaacgtaaatgcatgccgcttcgcctcgtccggcgtagaggatctgctcatgtttgacagcttatcatcgatgcataatgtgcctgtcaaatggacgaagcagggattctgcaaaccctatgctactccgtcaagccgtcaattgtctgattcgttaccaattatgacaacttgacggctacatcattcactttttcttcacaaccggcacggaactcgctcgggctggccccggtgcattttttaaatacccgcgagaaatagagttgatcgtcaaaaccaacattgcgaccgacggtggcgataggcatccgggtggtgctcaaaagcagcttcgcctggctgatacgttggtcctcgcgccagcttaagacgctaatccctaactgctggcggaaaagatgtgacagacgcgacggcgacaagcaaacatgctgtgcgacgctggcgatatcaaaattgctgtctgccaggtgatcgctgatgtactgacaagcctcgcgtacccgattatccatcggtggatggagcgactcgttaatcgcttccatgcgccgcagtaacaattgctcaagcagatttatcgccagcagctccgaatagcgcccttccccttgcccggcgttaatgatttgcccaaacaggtcgctgaaatgcggctggtgcgcttcatccgggcgaaagaaccccgtattggcaaatattgacggccagttaagccattcatgccagtaggcgcgcggacgaaagtaaacccactggtgataccattcgcgagcctccggatgacgaccgtagtgatgaatctctcctggcgggaacagcaaaatatcacccggtcggcaaacaaattctcgtccctgatttttcaccaccccctgaccgcgaatggtgagattgagaatataacctttcattcccagcggtcggtcgataaaaaaatcgagataaccgttggcctcaatcggcgttaaacccgccaccagatgggcattaaacgagtatcccggcagcaggggatcattttgcgcttcagccatacttttcatactcccgccattcagagaagaaaccaattgtccatattgcatcagacattgccgtcactgcgtcttttactggctcttctcgctaaccaaaccggtaaccccgcttattaaaagcattctgtaacaaagcgggaccaaagccatgacaaaaacgcgtaacaaaagtgtctataatcacggcagaaaagtccacattgattatttgcacggcgtcacactttgctatgccatagcatttttatccataagattagcggatcctacctgacgctttttatcgcaactctctactgtttctccatacccgtttttttgggctagcgaattcnnnnnnnnnnnnnnnnnnnnnnnnnnnnnnnatggatattaatactgaaactgagatcaagcaaaagcattcactaaccccctttcctgttttcctaatcagcccggcatttcgcgggcgatattttcacagctatttcaggagttcagccatgaacgcttattacattcaggatcgtcttgaggctcagagctgggcgcgtcactaccagcagctcgcccgtgaagagaaagaggcagaactggcagacgacatggaaaaaggcctgccccagcacctgtttgaatcgctatgcatcgatcatttgcaacgccacggggccagcaaaaaatccattacccgtgcgtttgatgacgatgttgagtttcaggagcgcatggcagaacacatccggtacatggttgaaaccattgctcaccaccaggttgatattgattcagaggtataattggctgttttggcggatgagagaagattttcagcggaaacacagaaaaaagcccgcacctgacagtgcgggctttttttttcgaccaaaggtccatgggtatggacagttttccctttgatatgtaacggtgaacagttgttctacttttgtttgttagtcttgatgcttcactgatagatacaagagccataagaacc